European Patent Application EP 4 733 400 A1, published April 29, 2026. Title: Antisense oligonucleotide targeting Hic-5. Applicant: Showa University. Application JP. The sequence listing filed with the application follows.

SEQUENCE LISTING (520 sequences)

SEQ ID NO: 1 - DNA, 16 bp, synthetic construct
  source 1..16: mol_type = other DNA
tgtgtgaagtggtggt

SEQ ID NO: 2 - DNA, 16 bp, synthetic construct
  source 1..16: mol_type = other DNA
atgtgtgaagtggtgg

SEQ ID NO: 3 - DNA, 16 bp, synthetic construct
  source 1..16: mol_type = other DNA
catgtgtgaagtggtg

SEQ ID NO: 4 - DNA, 14 bp, synthetic construct
  source 1..14: mol_type = other DNA
tggccatagggtgg

SEQ ID NO: 5 - DNA, 14 bp, synthetic construct
  source 1..14: mol_type = other DNA
gtggccatagggtg

SEQ ID NO: 6 - DNA, 16 bp, synthetic construct
  source 1..16: mol_type = other DNA
tgtgctgtatagatga

SEQ ID NO: 7 - DNA, 16 bp, synthetic construct
  source 1..16: mol_type = other DNA
aactgagacatgattt

SEQ ID NO: 8 - DNA, 16 bp, synthetic construct
  source 1..16: mol_type = other DNA
gaactgagacatgatt

SEQ ID NO: 9 - DNA, 16 bp, synthetic construct
  source 1..16: mol_type = other DNA
ggaactgagacatgat

SEQ ID NO: 10 - DNA, 16 bp, synthetic construct
  source 1..16: mol_type = other DNA
gggaactgagacatga

SEQ ID NO: 11 - DNA, 16 bp, synthetic construct
  source 1..16: mol_type = other DNA
tgggaactgagacatg

SEQ ID NO: 12 - DNA, 16 bp, synthetic construct
  source 1..16: mol_type = other DNA
atgggaactgagacat

SEQ ID NO: 13 - DNA, 16 bp, synthetic construct
  source 1..16: mol_type = other DNA
gatgggaactgagaca

SEQ ID NO: 14 - DNA, 16 bp, synthetic construct
  source 1..16: mol_type = other DNA
agatgggaactgagac

SEQ ID NO: 15 - DNA, 16 bp, synthetic construct
  source 1..16: mol_type = other DNA
tagatgggaactgaga

SEQ ID NO: 16 - DNA, 16 bp, synthetic construct
  source 1..16: mol_type = other DNA
gggtgagctcttgtct

SEQ ID NO: 17 - DNA, 16 bp, synthetic construct
  source 1..16: mol_type = other DNA
tgggtgagctcttgtc

SEQ ID NO: 18 - DNA, 16 bp, synthetic construct
  source 1..16: mol_type = other DNA
gtgggtgagctcttgt

SEQ ID NO: 19 - DNA, 16 bp, synthetic construct
  source 1..16: mol_type = other DNA
agtgggtgagctcttg

SEQ ID NO: 20 - DNA, 16 bp, synthetic construct
  source 1..16: mol_type = other DNA
cagtgggtgagctctt

SEQ ID NO: 21 - DNA, 16 bp, synthetic construct
  source 1..16: mol_type = other DNA
ctgaaggctttgaggg

SEQ ID NO: 22 - DNA, 16 bp, synthetic construct
  source 1..16: mol_type = other DNA
gctgaaggctttgagg

SEQ ID NO: 23 - DNA, 16 bp, synthetic construct
  source 1..16: mol_type = other DNA
ggctgaaggctttgag

SEQ ID NO: 24 - DNA, 16 bp, synthetic construct
  source 1..16: mol_type = other DNA
tggctgaaggctttga

SEQ ID NO: 25 - DNA, 16 bp, synthetic construct
  source 1..16: mol_type = other DNA
ttcctgagtggcggag

SEQ ID NO: 26 - DNA, 14 bp, synthetic construct
  source 1..14: mol_type = other DNA
tcctgagtggcgga

SEQ ID NO: 27 - DNA, 14 bp, synthetic construct
  source 1..14: mol_type = other DNA
ttcctgagtggcgg

SEQ ID NO: 28 - DNA, 16 bp, synthetic construct
  source 1..16: mol_type = other DNA
cagttcctgagtggcg

SEQ ID NO: 29 - DNA, 16 bp, synthetic construct
  source 1..16: mol_type = other DNA
ccagttcctgagtggc

SEQ ID NO: 30 - DNA, 16 bp, synthetic construct
  source 1..16: mol_type = other DNA
tccagttcctgagtgg

SEQ ID NO: 31 - DNA, 16 bp, synthetic construct
  source 1..16: mol_type = other DNA
atccagttcctgagtg

SEQ ID NO: 32 - DNA, 16 bp, synthetic construct
  source 1..16: mol_type = other DNA
tatccagttcctgagt

SEQ ID NO: 33 - DNA, 16 bp, synthetic construct
  source 1..16: mol_type = other DNA
ttgcccagctataggt

SEQ ID NO: 34 - DNA, 16 bp, synthetic construct
  source 1..16: mol_type = other DNA
cttgcccagctatagg

SEQ ID NO: 35 - DNA, 16 bp, synthetic construct
  source 1..16: mol_type = other DNA
acttgcccagctatag

SEQ ID NO: 36 - DNA, 16 bp, synthetic construct
  source 1..16: mol_type = other DNA
ttttgtgtcggatggg

SEQ ID NO: 37 - DNA, 16 bp, synthetic construct
  source 1..16: mol_type = other DNA
attttgtgtcggatgg

SEQ ID NO: 38 - DNA, 16 bp, synthetic construct
  source 1..16: mol_type = other DNA
cattttgtgtcggatg

SEQ ID NO: 39 - DNA, 16 bp, synthetic construct
  source 1..16: mol_type = other DNA
ccattttgtgtcggat

SEQ ID NO: 40 - DNA, 16 bp, synthetic construct
  source 1..16: mol_type = other DNA
accattttgtgtcgga

SEQ ID NO: 41 - DNA, 16 bp, synthetic construct
  source 1..16: mol_type = other DNA
agcatggaaatggttt

SEQ ID NO: 42 - DNA, 16 bp, synthetic construct
  source 1..16: mol_type = other DNA
gagcatggaaatggtt

SEQ ID NO: 43 - DNA, 16 bp, synthetic construct
  source 1..16: mol_type = other DNA
tgagcatggaaatggt

SEQ ID NO: 44 - DNA, 16 bp, synthetic construct
  source 1..16: mol_type = other DNA
ctgagcatggaaatgg

SEQ ID NO: 45 - DNA, 16 bp, synthetic construct
  source 1..16: mol_type = other DNA
gctgagcatggaaatg

SEQ ID NO: 46 - DNA, 16 bp, synthetic construct
  source 1..16: mol_type = other DNA
agcctttggtgagtgg

SEQ ID NO: 47 - DNA, 16 bp, synthetic construct
  source 1..16: mol_type = other DNA
gagcctttggtgagtg

SEQ ID NO: 48 - DNA, 16 bp, synthetic construct
  source 1..16: mol_type = other DNA
ggagcctttggtgagt

SEQ ID NO: 49 - DNA, 16 bp, synthetic construct
  source 1..16: mol_type = other DNA
aggagcctttggtgag

SEQ ID NO: 50 - DNA, 16 bp, synthetic construct
  source 1..16: mol_type = other DNA
aaggagcctttggtga

SEQ ID NO: 51 - DNA, 16 bp, synthetic construct
  source 1..16: mol_type = other DNA
ttttgaaggcttagtt

SEQ ID NO: 52 - DNA, 16 bp, synthetic construct
  source 1..16: mol_type = other DNA
tttttgaaggcttagt

SEQ ID NO: 53 - DNA, 16 bp, synthetic construct
  source 1..16: mol_type = other DNA
gtttttgaaggcttag

SEQ ID NO: 54 - DNA, 16 bp, synthetic construct
  source 1..16: mol_type = other DNA
tgtttttgaaggctta

SEQ ID NO: 55 - DNA, 16 bp, synthetic construct
  source 1..16: mol_type = other DNA
gtgtttttgaaggctt

SEQ ID NO: 56 - DNA, 14 bp, synthetic construct
  source 1..14: mol_type = other DNA
gcggacagcttggg

SEQ ID NO: 57 - DNA, 14 bp, synthetic construct
  source 1..14: mol_type = other DNA
ggcggacagcttgg

SEQ ID NO: 58 - DNA, 14 bp, synthetic construct
  source 1..14: mol_type = other DNA
tggcggacagcttg

SEQ ID NO: 59 - DNA, 14 bp, synthetic construct
  source 1..14: mol_type = other DNA
ctggcggacagctt

SEQ ID NO: 60 - DNA, 14 bp, synthetic construct
  source 1..14: mol_type = other DNA
gctggcggacagct

SEQ ID NO: 61 - DNA, 14 bp, synthetic construct
  source 1..14: mol_type = other DNA
tggcggtgcgctgg

SEQ ID NO: 62 - DNA, 14 bp, synthetic construct
  source 1..14: mol_type = other DNA
atggcggtgcgctg

SEQ ID NO: 63 - DNA, 14 bp, synthetic construct
  source 1..14: mol_type = other DNA
catggcggtgcgct

SEQ ID NO: 64 - DNA, 14 bp, synthetic construct
  source 1..14: mol_type = other DNA
ccatggcggtgcgc

SEQ ID NO: 65 - DNA, 14 bp, synthetic construct
  source 1..14: mol_type = other DNA
tccatggcggtgcg

SEQ ID NO: 66 - DNA, 14 bp, synthetic construct
  source 1..14: mol_type = other DNA
ctccatggcggtgc

SEQ ID NO: 67 - DNA, 14 bp, synthetic construct
  source 1..14: mol_type = other DNA
ggccatagggtggg

SEQ ID NO: 68 - DNA, 14 bp, synthetic construct
  source 1..14: mol_type = other DNA
ctgagtggcggagg

SEQ ID NO: 69 - DNA, 16 bp, synthetic construct
  source 1..16: mol_type = other DNA
agaggagaatggaggg

SEQ ID NO: 70 - DNA, 16 bp, synthetic construct
  source 1..16: mol_type = other DNA
aagaggagaatggagg

SEQ ID NO: 71 - DNA, 16 bp, synthetic construct
  source 1..16: mol_type = other DNA
gaagaggagaatggag

SEQ ID NO: 72 - DNA, 16 bp, synthetic construct
  source 1..16: mol_type = other DNA
gtcttttcttatcttc

SEQ ID NO: 73 - DNA, 16 bp, synthetic construct
  source 1..16: mol_type = other DNA
ggtcttttcttatctt

SEQ ID NO: 74 - DNA, 16 bp, synthetic construct
  source 1..16: mol_type = other DNA
gggtcttttcttatct

SEQ ID NO: 75 - DNA, 16 bp, synthetic construct
  source 1..16: mol_type = other DNA
tgggtcttttcttatc

SEQ ID NO: 76 - DNA, 16 bp, synthetic construct
  source 1..16: mol_type = other DNA
ctgggtcttttcttat

SEQ ID NO: 77 - DNA, 16 bp, synthetic construct
  source 1..16: mol_type = other DNA
gaagtcagagagtgag

SEQ ID NO: 78 - DNA, 16 bp, synthetic construct
  source 1..16: mol_type = other DNA
ggaagtcagagagtga

SEQ ID NO: 79 - DNA, 16 bp, synthetic construct
  source 1..16: mol_type = other DNA
cggaagtcagagagtg

SEQ ID NO: 80 - DNA, 16 bp, synthetic construct
  source 1..16: mol_type = other DNA
gcggaagtcagagagt

SEQ ID NO: 81 - DNA, 16 bp, synthetic construct
  source 1..16: mol_type = other DNA
cgcggaagtcagagag

SEQ ID NO: 82 - DNA, 16 bp, synthetic construct
  source 1..16: mol_type = other DNA
acgcggaagtcagaga

SEQ ID NO: 83 - DNA, 16 bp, synthetic construct
  source 1..16: mol_type = other DNA
aacgcggaagtcagag

SEQ ID NO: 84 - DNA, 16 bp, synthetic construct
  source 1..16: mol_type = other DNA
gaacgcggaagtcaga

SEQ ID NO: 85 - DNA, 16 bp, synthetic construct
  source 1..16: mol_type = other DNA
tgaacgcggaagtcag

SEQ ID NO: 86 - DNA, 16 bp, synthetic construct
  source 1..16: mol_type = other DNA
ttgaacgcggaagtca

SEQ ID NO: 87 - DNA, 16 bp, synthetic construct
  source 1..16: mol_type = other DNA
ccccagcatggtgtct

SEQ ID NO: 88 - DNA, 16 bp, synthetic construct
  source 1..16: mol_type = other DNA
tgcctcccagggcggt

SEQ ID NO: 89 - DNA, 16 bp, synthetic construct
  source 1..16: mol_type = other DNA
atgggctggttgcaga

SEQ ID NO: 90 - DNA, 16 bp, synthetic construct
  source 1..16: mol_type = other DNA
gatgggctggttgcag

SEQ ID NO: 91 - DNA, 16 bp, synthetic construct
  source 1..16: mol_type = other DNA
cgtggaaaccctcatc

SEQ ID NO: 92 - DNA, 16 bp, synthetic construct
  source 1..16: mol_type = other DNA
tcgtggaaaccctcat

SEQ ID NO: 93 - DNA, 16 bp, synthetic construct
  source 1..16: mol_type = other DNA
ctcgtggaaaccctca

SEQ ID NO: 94 - DNA, 16 bp, synthetic construct
  source 1..16: mol_type = other DNA
gctcgtggaaaccctc

SEQ ID NO: 95 - DNA, 14 bp, synthetic construct
  source 1..14: mol_type = other DNA
tcctccatggcggg

SEQ ID NO: 96 - DNA, 14 bp, synthetic construct
  source 1..14: mol_type = other DNA
gtcctccatggcgg

SEQ ID NO: 97 - DNA, 14 bp, synthetic construct
  source 1..14: mol_type = other DNA
ggtcctccatggcg

SEQ ID NO: 98 - DNA, 14 bp, synthetic construct
  source 1..14: mol_type = other DNA
cgcagggcgctctt

SEQ ID NO: 99 - DNA, 14 bp, synthetic construct
  source 1..14: mol_type = other DNA
ccgcagggcgctct

SEQ ID NO: 100 - DNA, 14 bp, synthetic construct
  source 1..14: mol_type = other DNA
tccgcagggcgctc

SEQ ID NO: 101 - DNA, 14 bp, synthetic construct
  source 1..14: mol_type = other DNA
ctccgcagggcgct

SEQ ID NO: 102 - DNA, 14 bp, synthetic construct
  source 1..14: mol_type = other DNA
cccagcatggtgtc

SEQ ID NO: 103 - DNA, 14 bp, synthetic construct
  source 1..14: mol_type = other DNA
ccccagcatggtgt

SEQ ID NO: 104 - DNA, 14 bp, synthetic construct
  source 1..14: mol_type = other DNA
gccccagcatggtg

SEQ ID NO: 105 - DNA, 14 bp, synthetic construct
  source 1..14: mol_type = other DNA
agccccagcatggt

SEQ ID NO: 106 - DNA, 14 bp, synthetic construct
  source 1..14: mol_type = other DNA
cccagggcggtgga

SEQ ID NO: 107 - DNA, 14 bp, synthetic construct
  source 1..14: mol_type = other DNA
tcccagggcggtgg

SEQ ID NO: 108 - DNA, 14 bp, synthetic construct
  source 1..14: mol_type = other DNA
ctcccagggcggtg

SEQ ID NO: 109 - DNA, 14 bp, synthetic construct
  source 1..14: mol_type = other DNA
atgggctggttgca

SEQ ID NO: 110 - DNA, 14 bp, synthetic construct
  source 1..14: mol_type = other DNA
gatgggctggttgc

SEQ ID NO: 111 - DNA, 14 bp, synthetic construct
  source 1..14: mol_type = other DNA
ctcgtggaaaccct

SEQ ID NO: 112 - DNA, 14 bp, synthetic construct
  source 1..14: mol_type = other DNA
gggtggaagcggcg

SEQ ID NO: 113 - DNA, 14 bp, synthetic construct
  source 1..14: mol_type = other DNA
cgggtggaagcggc

SEQ ID NO: 114 - DNA, 14 bp, synthetic construct
  source 1..14: mol_type = other DNA
ccgggtggaagcgg

SEQ ID NO: 115 - DNA, 14 bp, synthetic construct
  source 1..14: mol_type = other DNA
tccgggtggaagcg

SEQ ID NO: 116 - DNA, 14 bp, synthetic construct
  source 1..14: mol_type = other DNA
gtccgggtggaagc

SEQ ID NO: 117 - DNA, 14 bp, synthetic construct
  source 1..14: mol_type = other DNA
gcgcaggcagaagg

SEQ ID NO: 118 - DNA, 14 bp, synthetic construct
  source 1..14: mol_type = other DNA
ggcgcaggcagaag

SEQ ID NO: 119 - DNA, 14 bp, synthetic construct
  source 1..14: mol_type = other DNA
gggcgcaggcagaa

SEQ ID NO: 120 - DNA, 14 bp, synthetic construct
  source 1..14: mol_type = other DNA
cgggcgcaggcaga

SEQ ID NO: 121 - DNA, 14 bp, synthetic construct
  source 1..14: mol_type = other DNA
gcgggcgcaggcag

SEQ ID NO: 122 - DNA, 16 bp, synthetic construct
  source 1..16: mol_type = other DNA
accgaggcttgcatac

SEQ ID NO: 123 - DNA, 17 bp, synthetic construct
  source 1..17: mol_type = other DNA
ggcattaagttcctgaa

SEQ ID NO: 124 - DNA, 18 bp, synthetic construct
  source 1..18: mol_type = other DNA
tggcattaagttcctgaa

SEQ ID NO: 125 - DNA, 17 bp, synthetic construct
  source 1..17: mol_type = other DNA
tggcattaagttcctga

SEQ ID NO: 126 - DNA, 18 bp, synthetic construct
  source 1..18: mol_type = other DNA
gtggcattaagttcctga

SEQ ID NO: 127 - DNA, 18 bp, synthetic construct
  source 1..18: mol_type = other DNA
acatgatttcatctggag

SEQ ID NO: 128 - DNA, 18 bp, synthetic construct
  source 1..18: mol_type = other DNA
gacatgatttcatctgga

SEQ ID NO: 129 - DNA, 18 bp, synthetic construct
  source 1..18: mol_type = other DNA
agacatgatttcatctgg

SEQ ID NO: 130 - DNA, 18 bp, synthetic construct
  source 1..18: mol_type = other DNA
gaactgagacatgatttc

SEQ ID NO: 131 - DNA, 18 bp, synthetic construct
  source 1..18: mol_type = other DNA
ggaactgagacatgattt

SEQ ID NO: 132 - DNA, 18 bp, synthetic construct
  source 1..18: mol_type = other DNA
gggaactgagacatgatt

SEQ ID NO: 133 - DNA, 18 bp, synthetic construct
  source 1..18: mol_type = other DNA
tgggaactgagacatgat

SEQ ID NO: 134 - DNA, 18 bp, synthetic construct
  source 1..18: mol_type = other DNA
gatgggaactgagacatg

SEQ ID NO: 135 - DNA, 18 bp, synthetic construct
  source 1..18: mol_type = other DNA
agatgggaactgagacat

SEQ ID NO: 136 - DNA, 18 bp, synthetic construct
  source 1..18: mol_type = other DNA
ctagatgggaactgagac

SEQ ID NO: 137 - DNA, 18 bp, synthetic construct
  source 1..18: mol_type = other DNA
aggtttattgcaggagcc

SEQ ID NO: 138 - DNA, 18 bp, synthetic construct
  source 1..18: mol_type = other DNA
taggtttattgcaggagc

SEQ ID NO: 139 - DNA, 17 bp, synthetic construct
  source 1..17: mol_type = other DNA
aggtttattgcaggagc

SEQ ID NO: 140 - DNA, 18 bp, synthetic construct
  source 1..18: mol_type = other DNA
ataggtttattgcaggag

SEQ ID NO: 141 - DNA, 16 bp, synthetic construct
  source 1..16: mol_type = other DNA
cgctcgtggaaaccct

SEQ ID NO: 142 - DNA, 17 bp, synthetic construct
  source 1..17: mol_type = other DNA
cgctcgtggaaaccctc

SEQ ID NO: 143 - DNA, 18 bp, synthetic construct
  source 1..18: mol_type = other DNA
gcgctcaaagtagcactc

SEQ ID NO: 144 - DNA, 17 bp, synthetic construct
  source 1..17: mol_type = other DNA
cgctcaaagtagcactc

SEQ ID NO: 145 - DNA, 17 bp, synthetic construct
  source 1..17: mol_type = other DNA
gcgctcaaagtagcact

SEQ ID NO: 146 - DNA, 18 bp, synthetic construct
  source 1..18: mol_type = other DNA
agcgctcaaagtagcact

SEQ ID NO: 147 - DNA, 17 bp, synthetic construct
  source 1..17: mol_type = other DNA
agcgctcaaagtagcac

SEQ ID NO: 148 - DNA, 17 bp, synthetic construct
  source 1..17: mol_type = other DNA
agcgctcaaagtagcac

SEQ ID NO: 149 - DNA, 18 bp, synthetic construct
  source 1..18: mol_type = other DNA
gaagcgctcaaagtagca

SEQ ID NO: 150 - DNA, 17 bp, synthetic construct
  source 1..17: mol_type = other DNA
gaagcgctcaaagtagc

SEQ ID NO: 151 - DNA, 18 bp, synthetic construct
  source 1..18: mol_type = other DNA
gagaagcgctcaaagtag

SEQ ID NO: 152 - DNA, 17 bp, synthetic construct
  source 1..17: mol_type = other DNA
gagaagcgctcaaagta

SEQ ID NO: 153 - DNA, 18 bp, synthetic construct
  source 1..18: mol_type = other DNA
cagctgcaggaagtcccg

SEQ ID NO: 154 - DNA, 18 bp, synthetic construct
  source 1..18: mol_type = other DNA
ccgagatgtagttatcca

SEQ ID NO: 155 - DNA, 17 bp, synthetic construct
  source 1..17: mol_type = other DNA
ccgagatgtagttatcc

SEQ ID NO: 156 - DNA, 16 bp, synthetic construct
  source 1..16: mol_type = other DNA
ccgagatgtagttatc

SEQ ID NO: 157 - RNA, 16 nt, Mus musculus
  source 1..16: mol_type = transcribed RNA
accaccacttcacaca

SEQ ID NO: 158 - RNA, 16 nt, Mus musculus
  source 1..16: mol_type = transcribed RNA
ccaccacttcacacat

SEQ ID NO: 159 - RNA, 16 nt, Mus musculus
  source 1..16: mol_type = transcribed RNA
caccacttcacacatg

SEQ ID NO: 160 - RNA, 14 nt, Mus musculus
  source 1..14: mol_type = transcribed RNA
ccaccctatggcca

SEQ ID NO: 161 - RNA, 14 nt, Mus musculus
  source 1..14: mol_type = transcribed RNA
caccctatggccac

SEQ ID NO: 162 - RNA, 16 nt, Mus musculus
  source 1..16: mol_type = mRNA
tcatctatacagcaca

SEQ ID NO: 163 - RNA, 16 nt, Mus musculus
  source 1..16: mol_type = mRNA
aaatcatgtctcagtt

SEQ ID NO: 164 - RNA, 16 nt, Mus musculus
  source 1..16: mol_type = mRNA
aatcatgtctcagttc

SEQ ID NO: 165 - RNA, 16 nt, Mus musculus
  source 1..16: mol_type = mRNA
atcatgtctcagttcc

SEQ ID NO: 166 - RNA, 16 nt, Mus musculus
  source 1..16: mol_type = mRNA
tcatgtctcagttccc

SEQ ID NO: 167 - RNA, 16 nt, Mus musculus
  source 1..16: mol_type = mRNA
catgtctcagttccca

SEQ ID NO: 168 - RNA, 16 nt, Mus musculus
  source 1..16: mol_type = mRNA
atgtctcagttcccat

SEQ ID NO: 169 - RNA, 16 nt, Mus musculus
  source 1..16: mol_type = mRNA
tgtctcagttcccatc

SEQ ID NO: 170 - RNA, 16 nt, Mus musculus
  source 1..16: mol_type = mRNA
gtctcagttcccatct

SEQ ID NO: 171 - RNA, 16 nt, Mus musculus
  source 1..16: mol_type = mRNA
tctcagttcccatcta

SEQ ID NO: 172 - RNA, 16 nt, Mus musculus
  source 1..16: mol_type = mRNA
agacaagagctcaccc

SEQ ID NO: 173 - RNA, 16 nt, Mus musculus
  source 1..16: mol_type = mRNA
gacaagagctcaccca

SEQ ID NO: 174 - RNA, 16 nt, Mus musculus
  source 1..16: mol_type = mRNA
acaagagctcacccac

SEQ ID NO: 175 - RNA, 16 nt, Mus musculus
  source 1..16: mol_type = mRNA
caagagctcacccact

SEQ ID NO: 176 - RNA, 16 nt, Mus musculus
  source 1..16: mol_type = mRNA
aagagctcacccactg

SEQ ID NO: 177 - RNA, 16 nt, Mus musculus
  source 1..16: mol_type = mRNA
ccctcaaagccttcag

SEQ ID NO: 178 - RNA, 16 nt, Mus musculus
  source 1..16: mol_type = mRNA
cctcaaagccttcagc

SEQ ID NO: 179 - RNA, 16 nt, Mus musculus
  source 1..16: mol_type = mRNA
ctcaaagccttcagcc

SEQ ID NO: 180 - RNA, 16 nt, Mus musculus
  source 1..16: mol_type = mRNA
tcaaagccttcagcca

SEQ ID NO: 181 - RNA, 16 nt, Mus musculus
  source 1..16: mol_type = mRNA
ctccgccactcaggaa

SEQ ID NO: 182 - RNA, 14 nt, Mus musculus
  source 1..14: mol_type = mRNA
tccgccactcagga

SEQ ID NO: 183 - RNA, 14 nt, Mus musculus
  source 1..14: mol_type = mRNA
ccgccactcaggaa

SEQ ID NO: 184 - RNA, 16 nt, Mus musculus
  source 1..16: mol_type = mRNA
cgccactcaggaactg

SEQ ID NO: 185 - RNA, 16 nt, Mus musculus
  source 1..16: mol_type = mRNA
gccactcaggaactgg

SEQ ID NO: 186 - RNA, 16 nt, Mus musculus
  source 1..16: mol_type = mRNA
ccactcaggaactgga

SEQ ID NO: 187 - RNA, 16 nt, Mus musculus
  source 1..16: mol_type = mRNA
cactcaggaactggat

SEQ ID NO: 188 - RNA, 16 nt, Mus musculus
  source 1..16: mol_type = mRNA
actcaggaactggata

SEQ ID NO: 189 - RNA, 16 nt, Mus musculus
  source 1..16: mol_type = mRNA
acctatagctgggcaa

SEQ ID NO: 190 - RNA, 16 nt, Mus musculus
  source 1..16: mol_type = mRNA
cctatagctgggcaag

SEQ ID NO: 191 - RNA, 16 nt, Mus musculus
  source 1..16: mol_type = mRNA
ctatagctgggcaagt

SEQ ID NO: 192 - RNA, 16 nt, Mus musculus
  source 1..16: mol_type = mRNA
cccatccgacacaaaa

SEQ ID NO: 193 - RNA, 16 nt, Mus musculus
  source 1..16: mol_type = mRNA
ccatccgacacaaaat

SEQ ID NO: 194 - RNA, 16 nt, Mus musculus
  source 1..16: mol_type = mRNA
catccgacacaaaatg

SEQ ID NO: 195 - RNA, 16 nt, Mus musculus
  source 1..16: mol_type = mRNA
atccgacacaaaatgg

SEQ ID NO: 196 - RNA, 16 nt, Mus musculus
  source 1..16: mol_type = mRNA
tccgacacaaaatggt

SEQ ID NO: 197 - RNA, 16 nt, Mus musculus
  source 1..16: mol_type = mRNA
aaaccatttccatgct

SEQ ID NO: 198 - RNA, 16 nt, Mus musculus
  source 1..16: mol_type = mRNA
aaccatttccatgctc

SEQ ID NO: 199 - RNA, 16 nt, Mus musculus
  source 1..16: mol_type = mRNA
accatttccatgctca

SEQ ID NO: 200 - RNA, 16 nt, Mus musculus
  source 1..16: mol_type = mRNA
ccatttccatgctcag

SEQ ID NO: 201 - RNA, 16 nt, Mus musculus
  source 1..16: mol_type = mRNA
catttccatgctcagc

SEQ ID NO: 202 - RNA, 16 nt, Mus musculus
  source 1..16: mol_type = mRNA
ccactcaccaaaggct

SEQ ID NO: 203 - RNA, 16 nt, Mus musculus
  source 1..16: mol_type = mRNA
cactcaccaaaggctc

SEQ ID NO: 204 - RNA, 16 nt, Mus musculus
  source 1..16: mol_type = mRNA
actcaccaaaggctcc

SEQ ID NO: 205 - RNA, 16 nt, Mus musculus
  source 1..16: mol_type = mRNA
ctcaccaaaggctcct

SEQ ID NO: 206 - RNA, 16 nt, Mus musculus
  source 1..16: mol_type = mRNA
tcaccaaaggctcctt

SEQ ID NO: 207 - RNA, 16 nt, Mus musculus
  source 1..16: mol_type = mRNA
aactaagccttcaaaa

SEQ ID NO: 208 - RNA, 16 nt, Mus musculus
  source 1..16: mol_type = mRNA
actaagccttcaaaaa

SEQ ID NO: 209 - RNA, 16 nt, Mus musculus
  source 1..16: mol_type = mRNA
ctaagccttcaaaaac

SEQ ID NO: 210 - RNA, 16 nt, Mus musculus
  source 1..16: mol_type = mRNA
taagccttcaaaaaca

SEQ ID NO: 211 - RNA, 16 nt, Mus musculus
  source 1..16: mol_type = mRNA
aagccttcaaaaacac

SEQ ID NO: 212 - RNA, 14 nt, Mus musculus
  source 1..14: mol_type = mRNA
cccaagctgtccgc

SEQ ID NO: 213 - RNA, 14 nt, Mus musculus
  source 1..14: mol_type = mRNA
ccaagctgtccgcc

SEQ ID NO: 214 - RNA, 14 nt, Mus musculus
  source 1..14: mol_type = mRNA
caagctgtccgcca

SEQ ID NO: 215 - RNA, 14 nt, Mus musculus
  source 1..14: mol_type = mRNA
aagctgtccgccag

SEQ ID NO: 216 - RNA, 14 nt, Mus musculus
  source 1..14: mol_type = mRNA
agctgtccgccagc

SEQ ID NO: 217 - RNA, 14 nt, Mus musculus
  source 1..14: mol_type = mRNA
ccagcgcaccgcca

SEQ ID NO: 218 - RNA, 14 nt, Mus musculus
  source 1..14: mol_type = mRNA
cagcgcaccgccat

SEQ ID NO: 219 - RNA, 14 nt, Mus musculus
  source 1..14: mol_type = mRNA
agcgcaccgccatg

SEQ ID NO: 220 - RNA, 14 nt, Mus musculus
  source 1..14: mol_type = mRNA
gcgcaccgccatgg

SEQ ID NO: 221 - RNA, 14 nt, Mus musculus
  source 1..14: mol_type = mRNA
cgcaccgccatgga

SEQ ID NO: 222 - RNA, 14 nt, Mus musculus
  source 1..14: mol_type = mRNA
gcaccgccatggag

SEQ ID NO: 223 - RNA, 14 nt, Mus musculus
  source 1..14: mol_type = transcribed RNA
cccaccctatggcc

SEQ ID NO: 224 - RNA, 14 nt, Mus musculus
  source 1..14: mol_type = mRNA
cctccgccactcag

SEQ ID NO: 225 - RNA, 16 nt, Homo sapiens
  source 1..16: mol_type = mRNA
ccctccattctcctct

SEQ ID NO: 226 - RNA, 16 nt, Homo sapiens
  source 1..16: mol_type = mRNA
cctccattctcctctt

SEQ ID NO: 227 - RNA, 16 nt, Homo sapiens
  source 1..16: mol_type = mRNA
ctccattctcctcttc

SEQ ID NO: 228 - RNA, 16 nt, Homo sapiens
  source 1..16: mol_type = mRNA
gaagataagaaaagac

SEQ ID NO: 229 - RNA, 16 nt, Homo sapiens
  source 1..16: mol_type = mRNA
aagataagaaaagacc

SEQ ID NO: 230 - RNA, 16 nt, Homo sapiens
  source 1..16: mol_type = mRNA
agataagaaaagaccc

SEQ ID NO: 231 - RNA, 16 nt, Homo sapiens
  source 1..16: mol_type = mRNA
gataagaaaagaccca

SEQ ID NO: 232 - RNA, 16 nt, Homo sapiens
  source 1..16: mol_type = mRNA
ataagaaaagacccag

SEQ ID NO: 233 - RNA, 16 nt, Homo sapiens
  source 1..16: mol_type = mRNA
ctcactctctgacttc

SEQ ID NO: 234 - RNA, 16 nt, Homo sapiens
  source 1..16: mol_type = mRNA
tcactctctgacttcc

SEQ ID NO: 235 - RNA, 16 nt, Homo sapiens
  source 1..16: mol_type = mRNA
cactctctgacttccg

SEQ ID NO: 236 - RNA, 16 nt, Homo sapiens
  source 1..16: mol_type = mRNA
actctctgacttccgc

SEQ ID NO: 237 - RNA, 16 nt, Homo sapiens
  source 1..16: mol_type = mRNA
ctctctgacttccgcg

SEQ ID NO: 238 - RNA, 16 nt, Homo sapiens
  source 1..16: mol_type = mRNA
tctctgacttccgcgt

SEQ ID NO: 239 - RNA, 16 nt, Homo sapiens
  source 1..16: mol_type = mRNA
ctctgacttccgcgtt

SEQ ID NO: 240 - RNA, 16 nt, Homo sapiens
  source 1..16: mol_type = mRNA
tctgacttccgcgttc

SEQ ID NO: 241 - RNA, 16 nt, Homo sapiens
  source 1..16: mol_type = mRNA
ctgacttccgcgttca

SEQ ID NO: 242 - RNA, 16 nt, Homo sapiens
  source 1..16: mol_type = mRNA
tgacttccgcgttcaa

SEQ ID NO: 243 - RNA, 16 nt, Homo sapiens
  source 1..16: mol_type = mRNA
agacaccatgctgggg

SEQ ID NO: 244 - RNA, 16 nt, Homo sapiens
  source 1..16: mol_type = mRNA
accgccctgggaggca

SEQ ID NO: 245 - RNA, 16 nt, Homo sapiens
  source 1..16: mol_type = mRNA
tctgcaaccagcccat

SEQ ID NO: 246 - RNA, 16 nt, Homo sapiens
  source 1..16: mol_type = mRNA
ctgcaaccagcccatc

SEQ ID NO: 247 - RNA, 16 nt, Homo sapiens
  source 1..16: mol_type = mRNA
gatgagggtttccacg

SEQ ID NO: 248 - RNA, 16 nt, Homo sapiens
  source 1..16: mol_type = mRNA
atgagggtttccacga

SEQ ID NO: 249 - RNA, 16 nt, Homo sapiens
  source 1..16: mol_type = mRNA
tgagggtttccacgag

SEQ ID NO: 250 - RNA, 16 nt, Homo sapiens
  source 1..16: mol_type = mRNA
gagggtttccacgagc

SEQ ID NO: 251 - RNA, 14 nt, Homo sapiens
  source 1..14: mol_type = mRNA
cccgccatggagga

SEQ ID NO: 252 - RNA, 14 nt, Homo sapiens
  source 1..14: mol_type = mRNA
ccgccatggaggac

SEQ ID NO: 253 - RNA, 14 nt, Homo sapiens
  source 1..14: mol_type = mRNA
cgccatggaggacc

SEQ ID NO: 254 - RNA, 14 nt, Homo sapiens
  source 1..14: mol_type = mRNA
aagagcgccctgcg

SEQ ID NO: 255 - RNA, 14 nt, Homo sapiens
  source 1..14: mol_type = mRNA
agagcgccctgcgg

SEQ ID NO: 256 - RNA, 14 nt, Homo sapiens
  source 1..14: mol_type = mRNA
gagcgccctgcgga

SEQ ID NO: 257 - RNA, 14 nt, Homo sapiens
  source 1..14: mol_type = mRNA
agcgccctgcggag

SEQ ID NO: 258 - RNA, 14 nt, Homo sapiens
  source 1..14: mol_type = mRNA
gacaccatgctggg

SEQ ID NO: 259 - RNA, 14 nt, Homo sapiens
  source 1..14: mol_type = mRNA
acaccatgctgggg

SEQ ID NO: 260 - RNA, 14 nt, Homo sapiens
  source 1..14: mol_type = mRNA
caccatgctggggc

SEQ ID NO: 261 - RNA, 14 nt, Homo sapiens
  source 1..14: mol_type = mRNA
accatgctggggct

SEQ ID NO: 262 - RNA, 14 nt, Homo sapiens
  source 1..14: mol_type = mRNA
tccaccgccctggg

SEQ ID NO: 263 - RNA, 14 nt, Homo sapiens
  source 1..14: mol_type = mRNA
ccaccgccctggga

SEQ ID NO: 264 - RNA, 14 nt, Homo sapiens
  source 1..14: mol_type = mRNA
caccgccctgggag

SEQ ID NO: 265 - RNA, 14 nt, Homo sapiens
  source 1..14: mol_type = mRNA
tgcaaccagcccat

SEQ ID NO: 266 - RNA, 14 nt, Homo sapiens
  source 1..14: mol_type = mRNA
gcaaccagcccatc

SEQ ID NO: 267 - RNA, 14 nt, Homo sapiens
  source 1..14: mol_type = mRNA
agggtttccacgag

SEQ ID NO: 268 - RNA, 14 nt, Homo sapiens
  source 1..14: mol_type = mRNA
cgccgcttccaccc

SEQ ID NO: 269 - RNA, 14 nt, Homo sapiens
  source 1..14: mol_type = mRNA
gccgcttccacccg

SEQ ID NO: 270 - RNA, 14 nt, Homo sapiens
  source 1..14: mol_type = mRNA
ccgcttccacccgg

SEQ ID NO: 271 - RNA, 14 nt, Homo sapiens
  source 1..14: mol_type = mRNA
cgcttccacccgga

SEQ ID NO: 272 - RNA, 14 nt, Homo sapiens
  source 1..14: mol_type = mRNA
gcttccacccggac

SEQ ID NO: 273 - RNA, 14 nt, Homo sapiens
  source 1..14: mol_type = mRNA
ccttctgcctgcgc

SEQ ID NO: 274 - RNA, 14 nt, Homo sapiens
  source 1..14: mol_type = mRNA
cttctgcctgcgcc

SEQ ID NO: 275 - RNA, 14 nt, Homo sapiens
  source 1..14: mol_type = mRNA
ttctgcctgcgccc

SEQ ID NO: 276 - RNA, 14 nt, Homo sapiens
  source 1..14: mol_type = mRNA
tctgcctgcgcccg

SEQ ID NO: 277 - RNA, 14 nt, Homo sapiens
  source 1..14: mol_type = mRNA
ctgcctgcgcccgc

SEQ ID NO: 278 - RNA, 16 nt, Homo sapiens
  source 1..16: mol_type = mRNA
gtatgcaagcctcggt

SEQ ID NO: 279 - RNA, 17 nt, Homo sapiens
  source 1..17: mol_type = mRNA
ttcaggaacttaatgcc

SEQ ID NO: 280 - RNA, 18 nt, Homo sapiens
  source 1..18: mol_type = mRNA
ttcaggaacttaatgcca

SEQ ID NO: 281 - RNA, 17 nt, Homo sapiens
  source 1..17: mol_type = mRNA
tcaggaacttaatgcca

SEQ ID NO: 282 - RNA, 18 nt, Homo sapiens
  source 1..18: mol_type = mRNA
tcaggaacttaatgccac

SEQ ID NO: 283 - RNA, 18 nt, Homo sapiens
  source 1..18: mol_type = transcribed RNA
ctccagatgaaatcatgt

SEQ ID NO: 284 - RNA, 18 nt, Homo sapiens
  source 1..18: mol_type = transcribed RNA
tccagatgaaatcatgtc

SEQ ID NO: 285 - RNA, 18 nt, Homo sapiens
  source 1..18: mol_type = transcribed RNA
ccagatgaaatcatgtct

SEQ ID NO: 286 - RNA, 18 nt, Homo sapiens
  source 1..18: mol_type = mRNA
gaaatcatgtctcagttc

SEQ ID NO: 287 - RNA, 18 nt, Homo sapiens
  source 1..18: mol_type = mRNA
aaatcatgtctcagttcc

SEQ ID NO: 288 - RNA, 18 nt, Homo sapiens
  source 1..18: mol_type = mRNA
aatcatgtctcagttccc

SEQ ID NO: 289 - RNA, 18 nt, Homo sapiens
  source 1..18: mol_type = mRNA
atcatgtctcagttccca

SEQ ID NO: 290 - RNA, 18 nt, Homo sapiens
  source 1..18: mol_type = mRNA
catgtctcagttcccatc

SEQ ID NO: 291 - RNA, 18 nt, Homo sapiens
  source 1..18: mol_type = mRNA
atgtctcagttcccatct

SEQ ID NO: 292 - RNA, 18 nt, Homo sapiens
  source 1..18: mol_type = mRNA
gtctcagttcccatctag

SEQ ID NO: 293 - RNA, 18 nt, Homo sapiens
  source 1..18: mol_type = mRNA
ggctcctgcaataaacct

SEQ ID NO: 294 - RNA, 18 nt, Homo sapiens
  source 1..18: mol_type = mRNA
gctcctgcaataaaccta

SEQ ID NO: 295 - RNA, 17 nt, Homo sapiens
  source 1..17: mol_type = mRNA
gctcctgcaataaacct

SEQ ID NO: 296 - RNA, 18 nt, Homo sapiens
  source 1..18: mol_type = mRNA
ctcctgcaataaacctat

SEQ ID NO: 297 - RNA, 16 nt, Homo sapiens
  source 1..16: mol_type = mRNA
agggtttccacgagcg

SEQ ID NO: 298 - RNA, 17 nt, Homo sapiens
  source 1..17: mol_type = mRNA
gagggtttccacgagcg

SEQ ID NO: 299 - RNA, 18 nt, Homo sapiens
  source 1..18: mol_type = mRNA
gagtgctactttgagcgc

SEQ ID NO: 300 - RNA, 17 nt, Homo sapiens
  source 1..17: mol_type = mRNA
gagtgctactttgagcg

SEQ ID NO: 301 - RNA, 17 nt, Homo sapiens
  source 1..17: mol_type = mRNA
agtgctactttgagcgc

SEQ ID NO: 302 - RNA, 18 nt, Homo sapiens
  source 1..18: mol_type = mRNA
agtgctactttgagcgct

SEQ ID NO: 303 - RNA, 17 nt, Homo sapiens
  source 1..17: mol_type = mRNA
gtgctactttgagcgct

SEQ ID NO: 304 - RNA, 17 nt, Homo sapiens
  source 1..17: mol_type = mRNA
gtgctactttgagcgct

SEQ ID NO: 305 - RNA, 18 nt, Homo sapiens
  source 1..18: mol_type = mRNA
tgctactttgagcgcttc

SEQ ID NO: 306 - RNA, 17 nt, Homo sapiens
  source 1..17: mol_type = mRNA
gctactttgagcgcttc

SEQ ID NO: 307 - RNA, 18 nt, Homo sapiens
  source 1..18: mol_type = mRNA
ctactttgagcgcttctc

SEQ ID NO: 308 - RNA, 17 nt, Homo sapiens
  source 1..17: mol_type = mRNA
tactttgagcgcttctc

SEQ ID NO: 309 - RNA, 18 nt, Homo sapiens
  source 1..18: mol_type = mRNA
cgggacttcctgcagctg

SEQ ID NO: 310 - RNA, 18 nt, Homo sapiens
  source 1..18: mol_type = mRNA
tggataactacatctcgg

SEQ ID NO: 311 - RNA, 17 nt, Homo sapiens
  source 1..17: mol_type = mRNA
ggataactacatctcgg

SEQ ID NO: 312 - RNA, 16 nt, Homo sapiens
  source 1..16: mol_type = mRNA
gataactacatctcgg

SEQ ID NO: 313 - DNA, 16 bp, synthetic construct
  source 1..16: mol_type = other DNA
tgtgtgaagtggtggt

SEQ ID NO: 314 - DNA, 16 bp, synthetic construct
  source 1..16: mol_type = other DNA
atgtgtgaagtggtgg

SEQ ID NO: 315 - DNA, 16 bp, synthetic construct
  source 1..16: mol_type = other DNA
catgtgtgaagtggtg

SEQ ID NO: 316 - DNA, 14 bp, synthetic construct
  source 1..14: mol_type = other DNA
tggccatagggtgg

SEQ ID NO: 317 - DNA, 14 bp, synthetic construct
  source 1..14: mol_type = other DNA
gtggccatagggtg

SEQ ID NO: 318 - DNA, 16 bp, synthetic construct
  source 1..16: mol_type = other DNA
tgtgctgtatagatga

SEQ ID NO: 319 - DNA, 16 bp, synthetic construct
  source 1..16: mol_type = other DNA
aactgagacatgattt

SEQ ID NO: 320 - DNA, 16 bp, synthetic construct
  source 1..16: mol_type = other DNA
gaactgagacatgatt

SEQ ID NO: 321 - DNA, 16 bp, synthetic construct
  source 1..16: mol_type = other DNA
ggaactgagacatgat

SEQ ID NO: 322 - DNA, 16 bp, synthetic construct
  source 1..16: mol_type = other DNA
gggaactgagacatga

SEQ ID NO: 323 - DNA, 16 bp, synthetic construct
  source 1..16: mol_type = other DNA
tgggaactgagacatg

SEQ ID NO: 324 - DNA, 16 bp, synthetic construct
  source 1..16: mol_type = other DNA
atgggaactgagacat

SEQ ID NO: 325 - DNA, 16 bp, synthetic construct
  source 1..16: mol_type = other DNA
gatgggaactgagaca

SEQ ID NO: 326 - DNA, 16 bp, synthetic construct
  source 1..16: mol_type = other DNA
agatgggaactgagac

SEQ ID NO: 327 - DNA, 16 bp, synthetic construct
  source 1..16: mol_type = other DNA
tagatgggaactgaga

SEQ ID NO: 328 - DNA, 16 bp, synthetic construct
  source 1..16: mol_type = other DNA
gggtgagctcttgtct

SEQ ID NO: 329 - DNA, 16 bp, synthetic construct
  source 1..16: mol_type = other DNA
tgggtgagctcttgtc

SEQ ID NO: 330 - DNA, 16 bp, synthetic construct
  source 1..16: mol_type = other DNA
gtgggtgagctcttgt

SEQ ID NO: 331 - DNA, 16 bp, synthetic construct
  source 1..16: mol_type = other DNA
agtgggtgagctcttg

SEQ ID NO: 332 - DNA, 16 bp, synthetic construct
  source 1..16: mol_type = other DNA
cagtgggtgagctctt

SEQ ID NO: 333 - DNA, 16 bp, synthetic construct
  source 1..16: mol_type = other DNA
ctgaaggctttgaggg

SEQ ID NO: 334 - DNA, 16 bp, synthetic construct
  source 1..16: mol_type = other DNA
gctgaaggctttgagg

SEQ ID NO: 335 - DNA, 16 bp, synthetic construct
  source 1..16: mol_type = other DNA
ggctgaaggctttgag

SEQ ID NO: 336 - DNA, 16 bp, synthetic construct
  source 1..16: mol_type = other DNA
tggctgaaggctttga

SEQ ID NO: 337 - DNA, 16 bp, synthetic construct
  source 1..16: mol_type = other DNA
ttcctgagtggcggag

SEQ ID NO: 338 - DNA, 14 bp, synthetic construct
  source 1..14: mol_type = other DNA
tcctgagtggcgga

SEQ ID NO: 339 - DNA, 14 bp, synthetic construct
  source 1..14: mol_type = other DNA
ttcctgagtggcgg

SEQ ID NO: 340 - DNA, 16 bp, synthetic construct
  source 1..16: mol_type = other DNA
cagttcctgagtggcg

SEQ ID NO: 341 - DNA, 16 bp, synthetic construct
  source 1..16: mol_type = other DNA
ccagttcctgagtggc

SEQ ID NO: 342 - DNA, 16 bp, synthetic construct
  source 1..16: mol_type = other DNA
tccagttcctgagtgg

SEQ ID NO: 343 - DNA, 16 bp, synthetic construct
  source 1..16: mol_type = other DNA
atccagttcctgagtg

SEQ ID NO: 344 - DNA, 16 bp, synthetic construct
  source 1..16: mol_type = other DNA
tatccagttcctgagt

SEQ ID NO: 345 - DNA, 16 bp, synthetic construct
  source 1..16: mol_type = other DNA
ttgcccagctataggt

SEQ ID NO: 346 - DNA, 16 bp, synthetic construct
  source 1..16: mol_type = other DNA
cttgcccagctatagg

SEQ ID NO: 347 - DNA, 16 bp, synthetic construct
  source 1..16: mol_type = other DNA
acttgcccagctatag

SEQ ID NO: 348 - DNA, 16 bp, synthetic construct
  source 1..16: mol_type = other DNA
ttttgtgtcggatggg

SEQ ID NO: 349 - DNA, 16 bp, synthetic construct
  source 1..16: mol_type = other DNA
attttgtgtcggatgg

SEQ ID NO: 350 - DNA, 16 bp, synthetic construct
  source 1..16: mol_type = other DNA
cattttgtgtcggatg

SEQ ID NO: 351 - DNA, 16 bp, synthetic construct
  source 1..16: mol_type = other DNA
ccattttgtgtcggat

SEQ ID NO: 352 - DNA, 16 bp, synthetic construct
  source 1..16: mol_type = other DNA
accattttgtgtcgga

SEQ ID NO: 353 - DNA, 16 bp, synthetic construct
  source 1..16: mol_type = other DNA
agcatggaaatggttt

SEQ ID NO: 354 - DNA, 16 bp, synthetic construct
  source 1..16: mol_type = other DNA
gagcatggaaatggtt

SEQ ID NO: 355 - DNA, 16 bp, synthetic construct
  source 1..16: mol_type = other DNA
tgagcatggaaatggt

SEQ ID NO: 356 - DNA, 16 bp, synthetic construct
  source 1..16: mol_type = other DNA
ctgagcatggaaatgg

SEQ ID NO: 357 - DNA, 16 bp, synthetic construct
  source 1..16: mol_type = other DNA
gctgagcatggaaatg

SEQ ID NO: 358 - DNA, 16 bp, synthetic construct
  source 1..16: mol_type = other DNA
agcctttggtgagtgg

SEQ ID NO: 359 - DNA, 16 bp, synthetic construct
  source 1..16: mol_type = other DNA
gagcctttggtgagtg

SEQ ID NO: 360 - DNA, 16 bp, synthetic construct
  source 1..16: mol_type = other DNA
ggagcctttggtgagt

SEQ ID NO: 361 - DNA, 16 bp, synthetic construct
  source 1..16: mol_type = other DNA
aggagcctttggtgag

SEQ ID NO: 362 - DNA, 16 bp, synthetic construct
  source 1..16: mol_type = other DNA
aaggagcctttggtga

SEQ ID NO: 363 - DNA, 16 bp, synthetic construct
  source 1..16: mol_type = other DNA
ttttgaaggcttagtt

SEQ ID NO: 364 - DNA, 16 bp, synthetic construct
  source 1..16: mol_type = other DNA
tttttgaaggcttagt

SEQ ID NO: 365 - DNA, 16 bp, synthetic construct
  source 1..16: mol_type = other DNA
gtttttgaaggcttag

SEQ ID NO: 366 - DNA, 16 bp, synthetic construct
  source 1..16: mol_type = other DNA
tgtttttgaaggctta

SEQ ID NO: 367 - DNA, 16 bp, synthetic construct
  source 1..16: mol_type = other DNA
gtgtttttgaaggctt

SEQ ID NO: 368 - DNA, 14 bp, synthetic construct
  source 1..14: mol_type = other DNA
gcggacagcttggg

SEQ ID NO: 369 - DNA, 14 bp, synthetic construct
  source 1..14: mol_type = other DNA
ggcggacagcttgg

SEQ ID NO: 370 - DNA, 14 bp, synthetic construct
  source 1..14: mol_type = other DNA
tggcggacagcttg

SEQ ID NO: 371 - DNA, 14 bp, synthetic construct
  source 1..14: mol_type = other DNA
ctggcggacagctt

SEQ ID NO: 372 - DNA, 14 bp, synthetic construct
  source 1..14: mol_type = other DNA
gctggcggacagct

SEQ ID NO: 373 - DNA, 14 bp, synthetic construct
  source 1..14: mol_type = other DNA
tggcggtgcgctgg

SEQ ID NO: 374 - DNA, 14 bp, synthetic construct
  source 1..14: mol_type = other DNA
atggcggtgcgctg

SEQ ID NO: 375 - DNA, 14 bp, synthetic construct
  source 1..14: mol_type = other DNA
catggcggtgcgct

SEQ ID NO: 376 - DNA, 14 bp, synthetic construct
  source 1..14: mol_type = other DNA
ccatggcggtgcgc

SEQ ID NO: 377 - DNA, 14 bp, synthetic construct
  source 1..14: mol_type = other DNA
tccatggcggtgcg

SEQ ID NO: 378 - DNA, 14 bp, synthetic construct
  source 1..14: mol_type = other DNA
ctccatggcggtgc

SEQ ID NO: 379 - DNA, 14 bp, synthetic construct
  source 1..14: mol_type = other DNA
ggccatagggtggg

SEQ ID NO: 380 - DNA, 14 bp, synthetic construct
  source 1..14: mol_type = other DNA
ctgagtggcggagg

SEQ ID NO: 381 - DNA, 16 bp, synthetic construct
  source 1..16: mol_type = other DNA
agaggagaatggaggg

SEQ ID NO: 382 - DNA, 16 bp, synthetic construct
  source 1..16: mol_type = other DNA
aagaggagaatggagg

SEQ ID NO: 383 - DNA, 16 bp, synthetic construct
  source 1..16: mol_type = other DNA
gaagaggagaatggag

SEQ ID NO: 384 - DNA, 16 bp, synthetic construct
  source 1..16: mol_type = other DNA
gtcttttcttatcttc

SEQ ID NO: 385 - DNA, 16 bp, synthetic construct
  source 1..16: mol_type = other DNA
ggtcttttcttatctt

SEQ ID NO: 386 - DNA, 16 bp, synthetic construct
  source 1..16: mol_type = other DNA
gggtcttttcttatct

SEQ ID NO: 387 - DNA, 16 bp, synthetic construct
  source 1..16: mol_type = other DNA
tgggtcttttcttatc

SEQ ID NO: 388 - DNA, 16 bp, synthetic construct
  source 1..16: mol_type = other DNA
ctgggtcttttcttat

SEQ ID NO: 389 - DNA, 16 bp, synthetic construct
  source 1..16: mol_type = other DNA
gaagtcagagagtgag

SEQ ID NO: 390 - DNA, 16 bp, synthetic construct
  source 1..16: mol_type = other DNA
ggaagtcagagagtga

SEQ ID NO: 391 - DNA, 16 bp, synthetic construct
  source 1..16: mol_type = other DNA
cggaagtcagagagtg

SEQ ID NO: 392 - DNA, 16 bp, synthetic construct
  source 1..16: mol_type = other DNA
gcggaagtcagagagt

SEQ ID NO: 393 - DNA, 16 bp, synthetic construct
  source 1..16: mol_type = other DNA
cgcggaagtcagagag

SEQ ID NO: 394 - DNA, 16 bp, synthetic construct
  source 1..16: mol_type = other DNA
acgcggaagtcagaga

SEQ ID NO: 395 - DNA, 16 bp, synthetic construct
  source 1..16: mol_type = other DNA
aacgcggaagtcagag

SEQ ID NO: 396 - DNA, 16 bp, synthetic construct
  source 1..16: mol_type = other DNA
gaacgcggaagtcaga

SEQ ID NO: 397 - DNA, 16 bp, synthetic construct
  source 1..16: mol_type = other DNA
tgaacgcggaagtcag

SEQ ID NO: 398 - DNA, 16 bp, synthetic construct
  source 1..16: mol_type = other DNA
ttgaacgcggaagtca

SEQ ID NO: 399 - DNA, 16 bp, synthetic construct
  source 1..16: mol_type = other DNA
ccccagcatggtgtct

SEQ ID NO: 400 - DNA, 16 bp, synthetic construct
  source 1..16: mol_type = other DNA
tgcctcccagggcggt

SEQ ID NO: 401 - DNA, 16 bp, synthetic construct
  source 1..16: mol_type = other DNA
atgggctggttgcaga

SEQ ID NO: 402 - DNA, 16 bp, synthetic construct
  source 1..16: mol_type = other DNA
gatgggctggttgcag

SEQ ID NO: 403 - DNA, 16 bp, synthetic construct
  source 1..16: mol_type = other DNA
cgtggaaaccctcatc

SEQ ID NO: 404 - DNA, 16 bp, synthetic construct
  source 1..16: mol_type = other DNA
tcgtggaaaccctcat

SEQ ID NO: 405 - DNA, 16 bp, synthetic construct
  source 1..16: mol_type = other DNA
ctcgtggaaaccctca

SEQ ID NO: 406 - DNA, 16 bp, synthetic construct
  source 1..16: mol_type = other DNA
gctcgtggaaaccctc

SEQ ID NO: 407 - DNA, 14 bp, synthetic construct
  source 1..14: mol_type = other DNA
tcctccatggcggg

SEQ ID NO: 408 - DNA, 14 bp, synthetic construct
  source 1..14: mol_type = other DNA
gtcctccatggcgg

SEQ ID NO: 409 - DNA, 14 bp, synthetic construct
  source 1..14: mol_type = other DNA
ggtcctccatggcg

SEQ ID NO: 410 - DNA, 14 bp, synthetic construct
  source 1..14: mol_type = other DNA
cgcagggcgctctt

SEQ ID NO: 411 - DNA, 14 bp, synthetic construct
  source 1..14: mol_type = other DNA
ccgcagggcgctct

SEQ ID NO: 412 - DNA, 14 bp, synthetic construct
  source 1..14: mol_type = other DNA
tccgcagggcgctc

SEQ ID NO: 413 - DNA, 14 bp, synthetic construct
  source 1..14: mol_type = other DNA
ctccgcagggcgct

SEQ ID NO: 414 - DNA, 14 bp, synthetic construct
  source 1..14: mol_type = other DNA
cccagcatggtgtc

SEQ ID NO: 415 - DNA, 14 bp, synthetic construct
  source 1..14: mol_type = other DNA
ccccagcatggtgt

SEQ ID NO: 416 - DNA, 14 bp, synthetic construct
  source 1..14: mol_type = other DNA
gccccagcatggtg

SEQ ID NO: 417 - DNA, 14 bp, synthetic construct
  source 1..14: mol_type = other DNA
agccccagcatggt

SEQ ID NO: 418 - DNA, 14 bp, synthetic construct
  source 1..14: mol_type = other DNA
cccagggcggtgga

SEQ ID NO: 419 - DNA, 14 bp, synthetic construct
  source 1..14: mol_type = other DNA
tcccagggcggtgg

SEQ ID NO: 420 - DNA, 14 bp, synthetic construct
  source 1..14: mol_type = other DNA
ctcccagggcggtg

SEQ ID NO: 421 - DNA, 14 bp, synthetic construct
  source 1..14: mol_type = other DNA
atgggctggttgca

SEQ ID NO: 422 - DNA, 14 bp, synthetic construct
  source 1..14: mol_type = other DNA
gatgggctggttgc

SEQ ID NO: 423 - DNA, 14 bp, synthetic construct
  source 1..14: mol_type = other DNA
ctcgtggaaaccct

SEQ ID NO: 424 - DNA, 14 bp, synthetic construct
  source 1..14: mol_type = other DNA
gggtggaagcggcg

SEQ ID NO: 425 - DNA, 14 bp, synthetic construct
  source 1..14: mol_type = other DNA
cgggtggaagcggc

SEQ ID NO: 426 - DNA, 14 bp, synthetic construct
  source 1..14: mol_type = other DNA
ccgggtggaagcgg

SEQ ID NO: 427 - DNA, 14 bp, synthetic construct
  source 1..14: mol_type = other DNA
tccgggtggaagcg

SEQ ID NO: 428 - DNA, 14 bp, synthetic construct
  source 1..14: mol_type = other DNA
gtccgggtggaagc

SEQ ID NO: 429 - DNA, 14 bp, synthetic construct
  source 1..14: mol_type = other DNA
gcgcaggcagaagg

SEQ ID NO: 430 - DNA, 14 bp, synthetic construct
  source 1..14: mol_type = other DNA
ggcgcaggcagaag

SEQ ID NO: 431 - DNA, 14 bp, synthetic construct
  source 1..14: mol_type = other DNA
gggcgcaggcagaa

SEQ ID NO: 432 - DNA, 14 bp, synthetic construct
  source 1..14: mol_type = other DNA
cgggcgcaggcaga

SEQ ID NO: 433 - DNA, 14 bp, synthetic construct
  source 1..14: mol_type = other DNA
gcgggcgcaggcag

SEQ ID NO: 434 - DNA, 16 bp, synthetic construct
  source 1..16: mol_type = other DNA
accgaggcttgcatac

SEQ ID NO: 435 - DNA, 16 bp, synthetic construct
  source 1..16: mol_type = other DNA
accgaggcttgcatac

SEQ ID NO: 436 - DNA, 16 bp, synthetic construct
  source 1..16: mol_type = other DNA
accgaggcttgcatac

SEQ ID NO: 437 - DNA, 17 bp, synthetic construct
  source 1..17: mol_type = other DNA
ggcattaagttcctgaa

SEQ ID NO: 438 - DNA, 18 bp, synthetic construct
  source 1..18: mol_type = other DNA
tggcattaagttcctgaa

SEQ ID NO: 439 - DNA, 17 bp, synthetic construct
  source 1..17: mol_type = other DNA
tggcattaagttcctga

SEQ ID NO: 440 - DNA, 18 bp, synthetic construct
  source 1..18: mol_type = other DNA
gtggcattaagttcctga

SEQ ID NO: 441 - DNA, 18 bp, synthetic construct
  source 1..18: mol_type = other DNA
acatgatttcatctggag

SEQ ID NO: 442 - DNA, 18 bp, synthetic construct
  source 1..18: mol_type = other DNA
gacatgatttcatctgga

SEQ ID NO: 443 - DNA, 18 bp, synthetic construct
  source 1..18: mol_type = other DNA
agacatgatttcatctgg

SEQ ID NO: 444 - DNA, 18 bp, synthetic construct
  source 1..18: mol_type = other DNA
gaactgagacatgatttc

SEQ ID NO: 445 - DNA, 18 bp, synthetic construct
  source 1..18: mol_type = other DNA
ggaactgagacatgattt

SEQ ID NO: 446 - DNA, 18 bp, synthetic construct
  source 1..18: mol_type = other DNA
gggaactgagacatgatt

SEQ ID NO: 447 - DNA, 18 bp, synthetic construct
  source 1..18: mol_type = other DNA
tgggaactgagacatgat

SEQ ID NO: 448 - DNA, 18 bp, synthetic construct
  source 1..18: mol_type = other DNA
gatgggaactgagacatg

SEQ ID NO: 449 - DNA, 18 bp, synthetic construct
  source 1..18: mol_type = other DNA
agatgggaactgagacat

SEQ ID NO: 450 - DNA, 18 bp, synthetic construct
  source 1..18: mol_type = other DNA
ctagatgggaactgagac

SEQ ID NO: 451 - DNA, 18 bp, synthetic construct
  source 1..18: mol_type = other DNA
aggtttattgcaggagcc

SEQ ID NO: 452 - DNA, 18 bp, synthetic construct
  source 1..18: mol_type = other DNA
taggtttattgcaggagc

SEQ ID NO: 453 - DNA, 17 bp, synthetic construct
  source 1..17: mol_type = other DNA
aggtttattgcaggagc

SEQ ID NO: 454 - DNA, 18 bp, synthetic construct
  source 1..18: mol_type = other DNA
ataggtttattgcaggag

SEQ ID NO: 455 - DNA, 16 bp, synthetic construct
  source 1..16: mol_type = other DNA
gctcgtggaaaccctc

SEQ ID NO: 456 - DNA, 16 bp, synthetic construct
  source 1..16: mol_type = other DNA
gctcgtggaaaccctc

SEQ ID NO: 457 - DNA, 16 bp, synthetic construct
  source 1..16: mol_type = other DNA
gctcgtggaaaccctc

SEQ ID NO: 458 - DNA, 16 bp, synthetic construct
  source 1..16: mol_type = other DNA
gctcgtggaaaccctc

SEQ ID NO: 459 - DNA, 16 bp, synthetic construct
  source 1..16: mol_type = other DNA
gctcgtggaaaccctc

SEQ ID NO: 460 - DNA, 16 bp, synthetic construct
  source 1..16: mol_type = other DNA
cgctcgtggaaaccct

SEQ ID NO: 461 - DNA, 16 bp, synthetic construct
  source 1..16: mol_type = other DNA
cgctcgtggaaaccct

SEQ ID NO: 462 - DNA, 16 bp, synthetic construct
  source 1..16: mol_type = other DNA
cgctcgtggaaaccct

SEQ ID NO: 463 - DNA, 17 bp, synthetic construct
  source 1..17: mol_type = other DNA
cgctcgtggaaaccctc

SEQ ID NO: 464 - DNA, 17 bp, synthetic construct
  source 1..17: mol_type = other DNA
cgctcgtggaaaccctc

SEQ ID NO: 465 - DNA, 17 bp, synthetic construct
  source 1..17: mol_type = other DNA
cgctcgtggaaaccctc

SEQ ID NO: 466 - DNA, 18 bp, synthetic construct
  source 1..18: mol_type = other DNA
gcgctcaaagtagcactc

SEQ ID NO: 467 - DNA, 17 bp, synthetic construct
  source 1..17: mol_type = other DNA
cgctcaaagtagcactc

SEQ ID NO: 468 - DNA, 18 bp, synthetic construct
  source 1..18: mol_type = other DNA
gcgctcaaagtagcactc

SEQ ID NO: 469 - DNA, 17 bp, synthetic construct
  source 1..17: mol_type = other DNA
gcgctcaaagtagcact

SEQ ID NO: 470 - DNA, 18 bp, synthetic construct
  source 1..18: mol_type = other DNA
agcgctcaaagtagcact

SEQ ID NO: 471 - DNA, 17 bp, synthetic construct
  source 1..17: mol_type = other DNA
agcgctcaaagtagcac

SEQ ID NO: 472 - DNA, 17 bp, synthetic construct
  source 1..17: mol_type = other DNA
agcgctcaaagtagcac

SEQ ID NO: 473 - DNA, 18 bp, synthetic construct
  source 1..18: mol_type = other DNA
gaagcgctcaaagtagca

SEQ ID NO: 474 - DNA, 17 bp, synthetic construct
  source 1..17: mol_type = other DNA
gaagcgctcaaagtagc

SEQ ID NO: 475 - DNA, 18 bp, synthetic construct
  source 1..18: mol_type = other DNA
gagaagcgctcaaagtag

SEQ ID NO: 476 - DNA, 18 bp, synthetic construct
  source 1..18: mol_type = other DNA
gagaagcgctcaaagtag

SEQ ID NO: 477 - DNA, 18 bp, synthetic construct
  source 1..18: mol_type = other DNA
gagaagcgctcaaagtag

SEQ ID NO: 478 - DNA, 18 bp, synthetic construct
  source 1..18: mol_type = other DNA
gagaagcgctcaaagtag

SEQ ID NO: 479 - DNA, 18 bp, synthetic construct
  source 1..18: mol_type = other DNA
gagaagcgctcaaagtag

SEQ ID NO: 480 - DNA, 18 bp, synthetic construct
  source 1..18: mol_type = other DNA
gagaagcgctcaaagtag

SEQ ID NO: 481 - DNA, 17 bp, synthetic construct
  source 1..17: mol_type = other DNA
gagaagcgctcaaagta

SEQ ID NO: 482 - DNA, 18 bp, synthetic construct
  source 1..18: mol_type = other DNA
cagctgcaggaagtcccg

SEQ ID NO: 483 - DNA, 18 bp, synthetic construct
  source 1..18: mol_type = other DNA
ccgagatgtagttatcca

SEQ ID NO: 484 - DNA, 17 bp, synthetic construct
  source 1..17: mol_type = other DNA
ccgagatgtagttatcc

SEQ ID NO: 485 - DNA, 16 bp, synthetic construct
  source 1..16: mol_type = other DNA
ccgagatgtagttatc

SEQ ID NO: 486 - protein, 13 aa, synthetic construct
RRRRRRGGRRRRG

SEQ ID NO: 487 - RNA, 19 nt, synthetic construct
  source 1..19: mol_type = other RNA
ggaccagtctgaagataag

SEQ ID NO: 488 - RNA, 19 nt, synthetic construct
  source 1..19: mol_type = other RNA
cttatcttcagactggtcc

SEQ ID NO: 489 - RNA, 19 nt, synthetic construct
  source 1..19: mol_type = other RNA
ggaccagtctgaagataag

SEQ ID NO: 490 - RNA, 19 nt, synthetic construct
  source 1..19: mol_type = other RNA
cttatcttcagactggtcc

SEQ ID NO: 491 - DNA, 20 bp, synthetic construct
  source 1..20: mol_type = other DNA
gcaccgtcaaggctgagaac

SEQ ID NO: 492 - DNA, 19 bp, synthetic construct
  source 1..19: mol_type = other DNA
tggtgaagacgccagtgga

SEQ ID NO: 493 - DNA, 22 bp, synthetic construct
  source 1..22: mol_type = other DNA
agtgctactttgagcgcttctc

SEQ ID NO: 494 - DNA, 24 bp, synthetic construct
  source 1..24: mol_type = other DNA
gccgaagagcttcaggaagcaagg

SEQ ID NO: 495 - DNA, 21 bp, synthetic construct
  source 1..21: mol_type = other DNA
aggtcggtgtgaacggatttg

SEQ ID NO: 496 - DNA, 23 bp, synthetic construct
  source 1..23: mol_type = other DNA
tgtagaccatgtagttgaggtca

SEQ ID NO: 497 - DNA, 19 bp, synthetic construct
  source 1..19: mol_type = other DNA
atgtcacggttaggggctc

SEQ ID NO: 498 - DNA, 23 bp, synthetic construct
  source 1..23: mol_type = other DNA
ggcttgcatactgtgctgtatag

SEQ ID NO: 499 - DNA, 22 bp, synthetic construct
  source 1..22: mol_type = other DNA
ggtgaaggtcggagtcaacgga

SEQ ID NO: 500 - DNA, 22 bp, synthetic construct
  source 1..22: mol_type = other DNA
gagggatctcgctcctggaaga

SEQ ID NO: 501 - DNA, 20 bp, synthetic construct
  source 1..20: mol_type = other DNA
ccaggacagaccaacaaggg

SEQ ID NO: 502 - DNA, 20 bp, synthetic construct
  source 1..20: mol_type = other DNA
aaaagggagccccatccttc

SEQ ID NO: 503 - RNA, 1805 nt, Homo sapiens
  source 1..1805: mol_type = mRNA
gccctgttcgccccgcgccaccggcccgcgccccgccatggaggacctggatgccctgctctctgacctggagactaccacctcgcacatgccaaggtcaggggctcccaaagagcgccctgcggagcctctcacccctcccccatcctatggccaccagccacagacagggtctggggagtcttcaggagcctcgggggacaaggaccacctgtacagcacggtatgcaagcctcggtccccaaagcctgcagccccggcggcccctccattctcctcttccagcggtgtcttgggtaccgggctctgtgagctagatcggttgcttcaggaacttaatgccactcagttcaacatcacagatgaaatcatgtctcagttcccatctagcaaggtggcttcaggagagcagaaggaggaccagtctgaagataagaaaagacccagcctcccttccagcccgtctcctggcctcccaaaggcttctgccacctcagccactctggagctggatagactgatggcctcactctctgacttccgcgttcaaaaccatcttccagcctctgggccaactcagccaccggtggtgagctccacaaatgagggctccccatccccaccagagccgactggcaagggcagcctagacaccatgctggggctgctgcagtccgacctcagccgccggggtgttcccacccaggccaaaggcctctgtggctcctgcaataaacctattgctgggcaagtggtgacggctctgggccgcgcctggcaccccgagcacttcgtttgcggaggctgttccaccgccctgggaggcagcagcttcttcgagaaggatggagcccccttctgccccgagtgctactttgagcgcttctcgccaagatgtggcttctgcaaccagcccatccgacacaagatggtgaccgccttgggcactcactggcacccagagcatttctgctgcgtcagttgcggggagcccttcggagatgagggtttccacgagcgcgagggccgcccctactgccgccgggacttcctgcagctgttcgccccgcgctgccagggctgccagggccccatcctggataactacatctcggcgctcagcgcgctctggcacccggactgtttcgtctgcagggaatgcttcgcgcccttctcgggaggcagctttttcgagcacgagggccgcccgttgtgcgagaaccacttccacgcacgacgcggctcgctgtgcgccacgtgtggcctccctgtgaccggccgctgcgtgtcggccctgggtcgccgcttccacccggaccacttcacatgcaccttctgcctgcgcccgctcaccaaggggtccttccaggagcgcgccggcaagccctactgccagccctgcttcctgaagctcttcggctgacagcccgctcggctcgccctctcccccggaggccgcgccctcccggaaaagccgggtcctccagaccccgaggccttgctctcagagcgggaggccccacccactggagagccccgcccctaaggtactatgagtcctcaggggtcaagttcagaaacggcccagccagacctaaacccacacgcccacaaagtggattgcacacagacaagaactcccgtgcgggcctccactctattcccacccttgagggagcccccttactgggggagggtccttgcaattccagcgaatcggaggccaggccaggacgtccttgctccctgcaccctcactgttctgtgcactttttctacctacataaacacacgcattccacctc

SEQ ID NO: 504 - RNA, 5807 nt, Homo sapiens
  source 1..5807: mol_type = transcribed RNA
gccctgttcgccccgcgccaccggcccgcgccccgccatggaggacctgggtgagtggggccggatccccgggtccgtggcccctcaccgctgcccagagctgcctccccgccgtcgctctcccgcatctccccatccctgtcttcttacttctgcttttcgcctctgcccgcgcctcctttccaactccacgtcccccttcctgcctctcccttcctgcctttcctgggccggccgctccctcccttcttccctcgctgtgctcctccatcccaggctgcggcagatggaacgggaggtgcggcgcccgcgggcgcccgggcgcggggctctggggagggaggggttaaaggggcctcggcccggggaccgggaaagtagagggcacgggaaagtctggcatcaagttttggagaaaaaaagcgggcctgcctgcaccagagttttgggagaggaggagttaagggctcctgagcacagtgagggtcaggtccttgaggcaaggaagagaatagtaactcaggagtgcctaggcgcccgcgaaggcttcagggtttcacgcgggtgctcagagacgaagactgagggcaggacttctgggttctggaagtgaaagggctcaaaagacccggatctggggatgcagggatggagagaggtgtcttgtccggaagggggacccaggtatctcgtcctccctgcgaagcctggggctggaaggctgtgcgctccacgggagagaggggcttccggcccctggcggtagagggcgctgctcggtaggggtaactgacgctgtaccgcagataaacagccaatcagaaggcaggtcccagcgaagcgccagtgaggagcccagggcgggactcaggggcctgggagtggccaggctgggcggggcctgtgtaggtagagggaggagttaaccagcatggaagagagagcgtccaatcagaaagctgagggccaggcactgggccaatggagcaatttggaggggagccaaatttggcttgggtgaagagcccattttgactgcatcagagaagatggggagaataaaataatcaggaggctgggtttgtgcttggctccaagcgtgagcaactgggatattctggtcataaatattccttgctacccttcgagcagtgctctgcctggctctggccctgtgacctcttctcttaatactggcttctgtccttctccagtactgcccactgggaaccttatcttctgatctaaccgtgacccttgtctctctccctgatggcctcttcctgcagatgccctgctctctgacctggagactaccacctcgcacatgccaaggtcaggggctcccaaagagcgccctgcggagcctctcacccctcccccatcctatggccaccagccacaggtgagatcggatgttggggactggggcagccactagggccaggctcggcctggtctatggggatctcagcctcagtggggcagagtgcaggcctgtcatcccacctgtgcgtctccgctctgtagacagggtctggggagtcttcaggagcctcgggggacaaggaccacctgtacaggtgaggggcctggaaaccagggcatgggggccaactgagtctcaggtgaggaggcttggattccccacccctgaacccaggctcccactctgcttcccagcacggtatgcaagcctcggtccccaaagcctgcagccccggcggcccctccattctcctcttccagcggtgtcttgggtaccgggctctgtgagctagatcggttgcttcaggaacttaatgccactcagttcaacatcacaggtaccagggtgactgagagaggccttgatgcgataggggcaggggagggaagggtggggcagagactaagaggaatacacttcccagagtagcagttaaagggacctaaagcctcaagtgtgagggtgcgttgagcatggccctatatgtagcgtcctcctctcctctctccagatgaaatcatgtctcagttcccatctagcaaggtggcttcaggagagcagaaggaggaccagtctgaagataagaaaagacccagcctgtgagtttggcgtcgttgtcagggctgagagatgagtcctggatatctgagtcactagagggagcgttgctctgggaggctctgagatgacacaagcatgttcttcacagcccttccagcccgtctcctggcctcccaaaggcttctgccacctcagccactctggagctggatagactgatggcctcactctctgacttccgcgttcaaaaccatgtgagttgggcagtgggccagtgtccatttgtggctccccaaccccttctagacaattccacatctgctgctttgctgactcaattctcatgtcctccccgctgcagcttccagcctctgggccaactcagccaccggtggtgagctccacaaatgagggctccccatccccaccagagccgactggcaagggcagcctagacaccatgctggggctgctgcagtccgacctcagccgccggggtgttcccacccaggccaaaggcctctgtggctcctgcaataaacctattgctgggcaagtaagtggagccttgtgagaagggaggcagagacctgtcacagacccatctttagtgagagctgggctttatgctgttcccttttagtaagttaatctgggaagtgggtatcattattacttatgttttatggatgaggaaactgaagctctgaaccacacagcaggttagtggtagggtgaaaattccaaccatgttaccatttattgtggtcctactgtgtgccaggcactgtgccagctcctttacaaaccctcatctcatctgatcttcacaaaacactctgtggctccacccaatatctctcaggcatctacaaaggctctctcttcctccgtcagagtctggactgggttcactggtccttgttttattgactgagcagatgtgattgacaacagctgtgcctaggggttaacctagtgccccctgctagatcaagtacctgactcccagcccagaattgcccatctcagcaaaggagggtggcattgtgacttttgtggatcataggcactttcatcttcatgagtcccttcgtccattaaaataaatagatttttatgtctgtgttggtgtaaagatgggtatgttattattgtgtattacagcattttcttctagttcatttttttattctgaatttttaaaaacggatttttcacttcctccctcttatttattttgaggcaaattctcactcttgtgacccaagctggagtgcagtggtgcgattgtggctcactgcagcctcgaccttctgggctcaagtgatcctcccagctcagcctcccgagtagctgggactaaaggcgcccgccacctcgcccagctaattttatttatttattgtagagatggggcttcgccatgttgcccaggctggtctcaaactcctggactcaagtaatcctcccacctcagcctcccaaatgctaggattagaggcacgagccacccagcctgatcgtattttgattttaaaaaaattaaaacgtttttatgggcccctaaatgtattgtgggctccaggcgctgtgcctgctgtgcctcatgtataggtcaatcctggagcgcagctggaagacggaacacgggagctagatctccatcgcttacaggctgcgtgatctcgaacactggattctttattctgatcgctcagagaggactcgaaaaacgccgcgtaaatcttgcctcactgggcatgtggttgtcagagccgctctgacccgcctcacctcccactcgcaggtggtgacggctctgggccgcgcctggcaccccgagcacttcgtttgcggaggctgttccaccgccctgggaggcagcagcttcttcgagaaggatggagcccccttctgccccgagtgctactttgagcgcttctcgccaagatgtggcttctgcaaccagcccatccgacacgtgagccccgcccggccgcaccgagcccgccctatctcaccaggagagctgtgggacgggcctccaccgcatgggtcccgccccacccgcgataccccactccacccctaccccttccccttggcaatgtccacggccccttggactccactcttcctttctgacccccacgttcctagttagatcttctccccctccccccacgcatgccttagtccagtcacccgggttccgcgcgggagaggaaggcgcgaaggcacggaggccgcgctgagtgccctctccctccctgcagaagatggtgaccgccttgggcactcactggcacccagagcatttctgctgcgtcagttgcggggagcccttcggagatgagggtgagagtgaactcgactcccatcttaaaagctgcgggtcccctcgacgtctcgccccagcccctccgacctccggagtcctcagggccatggttttccttctgctctcttctggccctgccctctcctacacagactccggacccgagccctccccgctctgtcccgccatagacccggctcctccttccccaaggctccctcggactgcccctccttcggccccagatctcaggtcttgtgggtcccccgtcccgcccgcaccctttgctttcagcccactcggttccctctcctaggtttccacgagcgcgagggccgcccctactgccgccgggacttcctgcagctgttcgccccgcgctgccagggctgccagggccccatcctggataactacatctcggcgctcagcgcgctctggcacccggactgtttcgtctgcagggtgcgagctgcggggcggggcgttggaggggcgggtcaagggtacagggctgtggggcggggccttggaggggcgggtcaagggtgcagggcagggggcgggccctcgggggggcgggtcacgggaggtgctgctaggaacctcgggtggggcgagttttccgggcagggtcccaccggacgggattcttcgcgtctagggcgggctgcggggtcccagggcgttatccgctagtaacgcgcgttgtctggcagtggccgctgacctgtctgtcctctttcgcggcttcccttccccaggaatgcttcgcgcccttctcgggaggcagctttttcgagcacgagggccgcccgttgtgcgagaaccacttccacgcacgacgcggctcgctgtgcgccacgtgtggcctccctgtgaccggccgctgcgtgtcggccctgggtcgccgcttccacccggaccacttcacatgcaccttctgcctgcgcccgctcaccaaggggtccttccaggagcgcgccggcaagccctactgccagccctgcttcctgaagctcttcggctgacagcccgctcggctcgccctctcccccggaggccgcgccctcccggaaaagccgggtcctccagaccccgaggccttgctctcagagcgggaggccccacccactggagagccccgcccctaaggtactatgagtcctcaggggtcaagttcagaaacggcccagccagacctaaacccacacgcccacaaagtggattgcacacagacaagaactcccgtgcgggcctccactctattcccacccttgagggagcccccttactgggggagggtccttgcaattccagcgaatcggaggccaggccaggacgtccttgctccctgcaccctcactgttctgtgcactttttctacctacataaacacacgcattccacctc

SEQ ID NO: 505 - RNA, 3788 nt, Mus musculus
  source 1..3788: mol_type = mRNA
tcatgtctccatgctcccccttcatcgctccccccccccccactgtatcccagcgggtcccggcttccatacatggtcacggccctgcttctaactccctgacgtcccccccctccccgtcctccgcccccaccggacacggcccccgccctactctccccaagctgtccgccagcgcaccgccatggaggacctggacagggtctggagaatcttcaggaaccactggggacaaggatcatctatacagcacagtatgcaagcctcggtccccaaagcctgtggcccctgtggctcctccattctcctcttccagtggtgtgttgggcaatggcctctgtgagctagaccgtttgcttcaggaacttaatgccacccagttcaacattacagatgaaatcatgtctcagttcccatctagtaaaatggctgaaggggaagagaaggaggaccaatctgaagacaagagctcacccactgtccctcccagcccattccctgccccctcaaagccttcagccacctccgccactcaggaactggatagactgatggcctcgctctctgacttccgtgttcagaaccatcttccagcctcagggccacctcagcctccagcagcgagccccacccgtgaaggatgcccatctccaccaggacagactagcaaaggcagtctggacaccatgctgggcctgctgcagtctgacctcagccgtcgtggtgtccccacacaggccaaaggcctctgtggctcctgcaataaacctatagctgggcaagtggttacagccctgggcagagcctggcacccggagcacttcctttgcagcggttgttccacaaccctgggaggcagcagcttcttcgagaaggatggggctcccttttgccccgagtgctactttgagcgcttctccccacgatgtggcttctgtaaccaacccatccgacacaaaatggttaccgccttgggcacccactggcacccagaacatttctgctgcgtcagctgcggagagccttttggagaagagggtttccacgagcgggagggtcgtccgtactgccggcgggacttcctgcagctgttcgccccacgctgccagggctgccaaggccctattttggataactacatctcggcactcagcgcgctctggcacccagactgcttcgtgtgcagggaatgccttgcgcccttctccggaggcagcttttttgagcacgagggtcgccctttgtgtgaaaaccatttccatgctcagcgtggttcgctgtgtgccacgtgtggtctcccagtgaccggccgctgtgtgtccgctctgggccgacgcttccatccagaccacttcacctgcacattctgcctgcgcccactcaccaaaggctccttccaggagcgcgccagcaagccttactgccagccttgcttcctgaagctcttcggctgacctcctcttgggatcagagatctccaaaactaagccttcaaaaacacattcgtgaaaaagactgagtcctccagatccctggctctggagctacccaggcatccttgctccttctcccacccccatccccattgtggcccagccactggagaggcctacccctaagatgctctaggtttgtcaatttcagaaagggccccattagcctggaatgtagctctcactttgacatgattctggttctcttgtctgaccaagtagaggccaggatgtccctgttcacccatggcacactattctgtacacatttttttttctacaaacataaaaacacactccacactttacagtgccagagaaccttgctttactacccagagcccttgctctgtgctctgagggctccgggccacagctctggggaggggacagagctgcatccccttggggataacaataaatagcagatgaaggcaggcatggagaggtatgcctgtaatcccaacgcggaggccagggcagactatcttcagttgcatagcaaaattgaggtcagttgggttcaaaataaaacaaaaacccgcaaacccctggaaaccaaaattcaaagcaatggcaacagagggaaaggtgtagtacttcatgactctaatcgcagcatgccggaggcaagttcaacaccagttcaaaaacaggctggctgtgtatagtgagttccaggccagcctggctcttgggtataatagaagaccaagtaccaatagggtggggttggggcactagaagaccggggttcagttcctaacacctgcaattgtctgtaactccagttccaaggagtccaacacctcttctgacctctgtaggcaccaggtacacacatggtgcacagacatacatgcaggcaaaacgcccctacatataaagcacaatttttttttttaaaaaaaaggggggttggagaaatggttcagggtttgagtcctgtacattcagaagatgtgttcagtccccaaccccacatggtggctcccaatcacttgcaactccagttctgaggagttgaggacaccatgagttatcatttatcttaaaagacatttttaacataggttttaaccacagagtcaaaagagaggcactggggaagaaaggaagatatgcgtcaaaccataggtgtgggctcctgaaagacagacaaggcagctctgtcctagaggtgagtatataggattttaactgctaatgagtttctcaggcaccgtctacttctctgtctgtattcctctttttggtacttaagattgggtggacgtctggacaaagtgggagctacagaatgggaaaagatctttaccaattacacatccgatagagggtctatatcagtatgaaaagaactaaaatcaaacaaaaacctggatgttaagaaatcaaacagcccaattaaaaaagggcacagaactaagcaagttctcaaaagatgaaacacagtggctaagaaacatttaagggagtgagcagcatccttagtcatcagggaaatgcaaaccaaagctaccttgagcagcacttgggagggagacagagtcaggcctcctgatctgcagggtaagttccagaacagccagggctacacagagaaaccaacaaaaacaaatgaacaatcaaccccccccacacacacacagattacttggagatttcatcttactttaatcagaatggcaaagatcaataaaacaaatgacagcccatggcagtgggcatgtggggggaggggagcacttatgcgttgctgtgggagtgcagacttgtccagccactgtggaaatcagcgtggaggttcctcaggaatcagggaatagatagatctacctcacaatccagctgatcactcttgggcataccccaaaaggagtctacaccctactgtagagacacttgtccatccattgcagctctgttcaaagtatccaaaagctggaaatagcaaagatgctgttgatggatgaatggataaggaaaatatgttatatttacacaatggtatattattcagctgtttaaaaacatgcaataatgaaattcaccagtaaatggatggaactagaaaaaaataattctgagcaagcaaattcagatccagaaagacaaacgtggtatgtattctcctatgtgtggatgttagcttttaagctctcaatagacatgctacaatccatataatcacagaggttagatatggagtaagggacttgccgggtagattgtacaaggaaggggaaatagaatatatatagttatggagagacaggagaacaggaagattac

SEQ ID NO: 506 - RNA, 8888 nt, Mus musculus
  source 1..8888: mol_type = transcribed RNA
tcatgtctccatgctcccccttcatcgctccccccccccccactgtatcccagcgggtcccggcttccatacatggtcacggccctgcttctaactccctgacgtcccccccctccccgtcctccgcccccaccggacacggcccccgccctactctccccaagctgtccgccagcgcaccgccatggaggacctgggtgagtgaggagatccccctagcctctcatccttccccgcatctatccccttcccaactcacacttcttccccatctcagctttctctctccattttctcgcctcagcctgcctgtgcctccctcccaaatccacataccctttcctgcctctccctttcctgcctcgcttgcgacaagccgctccctccgttcttccctggctctctctgctcactcaatcctgcttgtgcaatggacaaagtgttgaggcacccacgggggcctggattcagagactctgggtaggaaggggttaagagatcactgagtcccgggactgggaaaatagactagagaggagagtgtgacctggagtttcggagatgaaaaggacctatatcagggtttcaagaagagttgagtgctcccaggtagagcagaggtcaagaaagtcctcagggcaagaaagagaataatagagaatgccagggttatagaaagaagtctaaggcttctaccgtagaggctcggagaagagtaaagggacggggcgtagataaagcgccccaggcatctcgtcccctctattcgcctaggctgagactagaagactctgctcttcgtggcagaatttctagatccagcagcagagggcgctcgtcaataatagtacatggataagacgtacaccaaaaagccgctccctgccagggccacttaaaggacagggctagacttcagtgtggccaagtggaccaagctggggagaagtagtaagtatgtcacagcaaacatctaatcaggaagttgggtgtcaaacatacagccgattgaacaatttgggtacagtaagagacaatctgggctgcaccagaaaagatggagagaataaaagatcattagttggtttgtacttggctcccagggtaagtcaagggagaggtctgatcataaataccccgccaccccatccctccccctccgcccctccatccccactccccccgcgctactattctacttttttgccttggtctgaccctgtgagtatggttttggccgctgcctttaacaccggctttctaccttttaaaacacggacacttgaaatcctttatactctaacctcttaagaccttgacatcccctccttcccaaactctcaccctgagggcctctcaccacagatgccctgctctctgacctggagaccaccacttcacacatgtcacggttaggggctccaaaagagcgcccaccagagacactcacacctcccccaccctatggccaccagccacaggtgagatgagattttgggttctgggggtagccattagggcctgggttggtctgggctaggggacatcagagtctgagtgaggcaaggaacatgactgtccttccacaaatacctctactctctatagacagggtctggagaatcttcaggaaccactggggacaaggatcatctatacaggtgaggggcctgggaactgggctaggaagatggggaagccagtttcagttcagaggaggggactcggattccctaccctaaacccaggttccctcctgcccttagcacagtatgcaagcctcggtccccaaagcctgtggcccctgtggctcctccattctcctcttccagtggtgtgttgggcaatggcctctgtgagctagaccgtttgcttcaggaacttaatgccacccagttcaacattacaggtaccagggttaccgagacagtcttggatggcttggggacagggcaaagaagggcagagtctaagggactcaaactgtccgaggagccattaaaggacgggaagccttcactgggagggtggactgatatgggctccttgccagtgttgttctctcatctctccagatgaaatcatgtctcagttcccatctagtaaaatggctgaaggggaagagaaggaggaccaatctgaagacaagagctcacccactgtgtgagtttggtagagtgggcagggctgggaagcggatgatgggtcctgcatgcctgacttaccagaggggtgttaggctggcaggttctgaggtgattcacggtgtcctccacagccctcccagcccattccctgccccctcaaagccttcagccacctccgccactcaggaactggatagactgatggcctcgctctctgacttccgtgttcagaaccatgtgagtctgcaaggattttggtccgtgtcactttgtggctcaccaatccagtcgtgatgcttccagtctgtggctttgttgactcagtgtcctctttactgcagcttccagcctcagggccacctcagcctccagcagcgagccccacccgtgaaggatgcccatctccaccaggacagactagcaaaggcagtctggacaccatgctgggcctgctgcagtctgacctcagccgtcgtggtgtccccacacaggccaaaggcctctgtggctcctgcaataaacctatagctgggcaagtaagttcagtaccttgagcagtggcatatactcacatatccacctttaagaatcagactggcgtggtggtgcacaccattaaccccagcactcaggaggcagaggcaggcggatttctgagttcgaggccagcctggtctacaaagtgagttccagggacagccagggctatacagagaaaccctgtctcgaaaaaaccaaaaacaaacaaacaaaaaaaagaatcagactttgtggtttttcccttttaaaatgtttcctcactctttgagaatttaatgcatgtacaggttagatacaaagtgagattcgtgttagatacaatgtatcttaacaccttcctctatttcttccagtgcccctttatattcccaacttcatgtcatcttttttttttttttttaaaaaaagtctaccaggtacagttagtgcttccagtgtgtgaatgggtgtagggccatcctttggagcactggcccctgccaggggctacatccctgaagaaaacaagtgccgtcacctaggagccaacaactgccaatcactcctcagctaggggaagggctaaatgagccccttcctcattcttgctggaattttgactggctccatactgtgtaggtctcatgaaggatctacagctcatgagcgtgtgagtgcaccagccaggcatgctgagaaagcacagcttcacagctgtcaacctctggctcttacaacctggccacgccctgttccgtgatgctcgctgagccttgtggggacactgtgggagataaatgctccaattaggactgtgtgtttgcccctttcaatgagtatcttgaaatggaatttgtttttccttgtgatgttgaggccagaacttagacccttgcatttgttagatagacttcccctcactaagctttgccctaactcttgggacaggtgtactggaattatagggatgcacggccccttcccaggttatatgtaattcttggagattgaatccaagactgtgtgtgtgctaagtgatcagtctaccacctctagcccaacccttgggattttgagacaaggtcttatgtactatgtagcacaggctgccctaaaacccatgattgtgccccctttacctcccaagttctagaaattttagcatgtgctactatgcccacctgaaatggacattattatttatattttatgtgttttttgaaaaaaaatttgagggagtgtctcactgtaacctaggttgaccagaagctcactctgtagcccagactggccttgaactcagggctatcatcgtcctcctcaagccttctaagtgctggatgtacaggagtgagccaccatgcccagctatggtttatgtttccttccttccttccttccttccttccttccttccttccttccttctttctctctctccctctttctttctccctctctttctttctccctccctttctttctccctctctttctttctccctccctccttctctttctttctttctttctttctttctttttctttctttctttcttccttccttccttccttccttccttccttccttcctttctttctaaaatgtgcattggtgttttccctgagttaataggctcagctgccatgtaggtgctgggaatagaactcaggtcttctggaagagaagccagtgcttttaaccactgaaccatctctcccagccccctattttatgttttcttaatttgaaaagttgcgtgtgtgctagggactaaagctggggttttatgcatgctaagcacacctttaccattgaatactcctagcaccatgtatatttatgaatgagaaaacggaaactcttagtgataagccataaggtaagaactccaacctgtttagtatttggtgtggccctactgtgtgctgaccactgtactagttctttttcaaacccctatttcatttaatcttcccaaagggctcattagttttgcttggtatctctcgggaatcataaaaactgtctctctttcctttctggtccagaagtcctgcttcttggatcatggatcaaggtgtgacctctgtgaggctctaggtactccagacttcatgggagcttcctctactaaaactcactctgtatcggcataaagaggactctgttttctagcgtggtgcctaaatagactttaaagtaactaaacctttcgtgggcccttagaaggagtgtggcccagatacaccactatgccttgcgtgcttgtaagcctgagggtaaacctgtaaggccagccctggacctctaacacagtttgtagagacttggacacttgggtttgttgttatttgtttgtttgtttgtttgtttcatcctgatcaccctgctttctgaggttggcaagtctggtttgagagtcaggaacttagtctatcaagatgctttaagccaacccagcacaaatattctggatcatatctgcttaattttccgttaagactgggaaaatgccaggtatataaaccttagctcgtccagctcctgccaggtggagagccaatctgacagaaacctcctgttcaacttggcaggtggttacagccctgggcagagcctggcacccggagcacttcctttgcagcggttgttccacaaccctgggaggcagcagcttcttcgagaaggatggggctcccttttgccccgagtgctactttgagcgcttctccccacgatgtggcttctgtaaccaacccatccgacacgtaagctctgcagacctccaccgattaacctgtttcagagaggactggccatatggagacctatctcttccacctacctccacgcccaccctaccctgtctcttcagtttttcctctttagccccaaatcctttgttagttctcccgccttccctgggttcccagagggaagtggagggaagaagggagaagaggtgacaatagtgtcctttttccgttttatgcagaaaatggttaccgccttgggcacccactggcacccagaacatttctgctgcgtcagctgcggagagccttttggagaagagggtgagagctgaaacttaaaagctacaggtccacttttctcctccccataagttttcttcaattccatctggcctttccatccgtgggtcccaactcccgcctctatccccacccaccgcgcccctttccctgtcctagaccctatccttccctccctgttctgcatacccactgccacgctttgatcttgtagtcccgcccacaccgtctgtctccgcccccaggtttccacgagcgggagggtcgtccgtactgccggcgggacttcctgcagctgttcgccccacgctgccagggctgccaaggccctattttggataactacatctcggcactcagcgcgctctggcacccagactgcttcgtgtgcagggtgcgtggctgtggggagcgggctaggagcccagggtgtgatgattcgttgattagtcgcttcacttttgctgcaaagctgcaggagtcagggtggatgctagttatccacacgggttacctggttagggttttggcttatttttgttaattcttccttctggtaggaatgccttgcgcccttctccggaggcagcttttttgagcacgagggtcgccctttgtgtgaaaaccatttccatgctcagcgtggttcgctgtgtgccacgtgtggtctcccagtgaccggccgctgtgtgtccgctctgggccgacgcttccatccagaccacttcacctgcacattctgcctgcgcccactcaccaaaggctccttccaggagcgcgccagcaagccttactgccagccttgcttcctgaagctcttcggctgacctcctcttgggatcagagatctccaaaactaagccttcaaaaacacattcgtgaaaaagactgagtcctccagatccctggctctggagctacccaggcatccttgctccttctcccacccccatccccattgtggcccagccactggagaggcctacccctaagatgctctaggtttgtcaatttcagaaagggccccattagcctggaatgtagctctcactttgacatgattctggttctcttgtctgaccaagtagaggccaggatgtccctgttcacccatggcacactattctgtacacatttttttttctacaaacataaaaacacactccacactttacagtgccagagaaccttgctttactacccagagcccttgctctgtgctctgagggctccgggccacagctctggggaggggacagagctgcatccccttggggataacaataaatagcagatgaaggcaggcatggagaggtatgcctgtaatcccaacgcggaggccagggcagactatcttcagttgcatagcaaaattgaggtcagttgggttcaaaataaaacaaaaacccgcaaacccctggaaaccaaaattcaaagcaatggcaacagagggaaaggtgtagtacttcatgactctaatcgcagcatgccggaggcaagttcaacaccagttcaaaaacaggctggctgtgtatagtgagttccaggccagcctggctcttgggtataatagaagaccaagtaccaatagggtggggttggggcactagaagaccggggttcagttcctaacacctgcaattgtctgtaactccagttccaaggagtccaacacctcttctgacctctgtaggcaccaggtacacacatggtgcacagacatacatgcaggcaaaacgcccctacatataaagcacaatttttttttttaaaaaaaaggggggttggagaaatggttcagggtttgagtcctgtacattcagaagatgtgttcagtccccaaccccacatggtggctcccaatcacttgcaactccagttctgaggagttgaggacaccatgagttatcatttatcttaaaagacatttttaacataggttttaaccacagagtcaaaagagaggcactggggaagaaaggaagatatgcgtcaaaccataggtgtgggctcctgaaagacagacaaggcagctctgtcctagaggtgagtatataggattttaactgctaatgagtttctcaggcaccgtctacttctctgtctgtattcctctttttggtacttaagattgggtggacgtctggacaaagtgggagctacagaatgggaaaagatctttaccaattacacatccgatagagggtctatatcagtatgaaaagaactaaaatcaaacaaaaacctggatgttaagaaatcaaacagcccaattaaaaaagggcacagaactaagcaagttctcaaaagatgaaacacagtggctaagaaacatttaagggagtgagcagcatccttagtcatcagggaaatgcaaaccaaagctaccttgagcagcacttgggagggagacagagtcaggcctcctgatctgcagggtaagttccagaacagccagggctacacagagaaaccaacaaaaacaaatgaacaatcaaccccccccacacacacacagattacttggagatttcatcttactttaatcagaatggcaaagatcaataaaacaaatgacagcccatggcagtgggcatgtggggggaggggagcacttatgcgttgctgtgggagtgcagacttgtccagccactgtggaaatcagcgtggaggttcctcaggaatcagggaatagatagatctacctcacaatccagctgatcactcttgggcataccccaaaaggagtctacaccctactgtagagacacttgtccatccattgcagctctgttcaaagtatccaaaagctggaaatagcaaagatgctgttgatggatgaatggataaggaaaatatgttatatttacacaatggtatattattcagctgtttaaaaacatgcaataatgaaattcaccagtaaatggatggaactagaaaaaaataattctgagcaagcaaattcagatccagaaagacaaacgtggtatgtattctcctatgtgtggatgttagcttttaagctctcaatagacatgctacaatccatataatcacagaggttagatatggagtaagggacttgccgggtagattgtacaaggaaggggaaatagaatatatatagttatggagagacaggagaacaggaagattac

SEQ ID NO: 507 - DNA, 22 bp, synthetic construct
  source 1..22: mol_type = other DNA
agacatgttcagctttgtggac

SEQ ID NO: 508 - DNA, 19 bp, synthetic construct
  source 1..19: mol_type = other DNA
gcagctgacttcagggatg

SEQ ID NO: 509 - DNA, 19 bp, synthetic construct
  source 1..19: mol_type = other DNA
acccgatggcaacaatgga

SEQ ID NO: 510 - DNA, 20 bp, synthetic construct
  source 1..20: mol_type = other DNA
accagcagggccttgttcac

SEQ ID NO: 511 - DNA, 20 bp, synthetic construct
  source 1..20: mol_type = other DNA
tcttctgctgcgtgacaacc

SEQ ID NO: 512 - DNA, 21 bp, synthetic construct
  source 1..21: mol_type = other DNA
gagaaaccagcttggaaccag

SEQ ID NO: 513 - DNA, 19 bp, synthetic construct
  source 1..19: mol_type = other DNA
gagtgctattgcgcttccc

SEQ ID NO: 514 - DNA, 19 bp, synthetic construct
  source 1..19: mol_type = other DNA
ggttgccgaagtcacaggt

SEQ ID NO: 515 - DNA, 23 bp, synthetic construct
  source 1..23: mol_type = other DNA
attaaccccaactatgaagtgcc

SEQ ID NO: 516 - DNA, 21 bp, synthetic construct
  source 1..21: mol_type = other DNA
ctgtctcctcactgaaggctc

SEQ ID NO: 517 - DNA, 20 bp, synthetic construct
  source 1..20: mol_type = other DNA
cgctcgtggaaaccctcatc

SEQ ID NO: 518 - DNA, 20 bp, synthetic construct
  source 1..20: mol_type = other DNA
gcgctcgtggaaaccctcat

SEQ ID NO: 519 - DNA, 20 bp, synthetic construct
  source 1..20: mol_type = other DNA
cgcgctcgtggaaaccctca

SEQ ID NO: 520 - DNA, 20 bp, synthetic construct
  source 1..20: mol_type = other DNA
tcgcgctcgtggaaaccctc